European Patent Application EP 4 722 373 A1, published April 8, 2026. Title: 一种腺病毒载体疫苗及其制备方法和应用. Applicant: 康希诺生物股份公司. The sequence listing filed with the application follows.

SEQUENCE LISTING (50 sequences)

SEQ ID NO: 1 - protein, 942 aa, synthetic construct
MATPSMLPQWAYMHIAGQDASEYLSPGLVQFARATDTYFSLGNKFRNPTVAPTHDVTTDRSQRLTLRFVPVDREDNTYSYKVRYTLAVGDNRVLDMASTYFDIRGVLDRGPSFKPYSGTAYNSLAPKGAPNSSQWEQKKAGNGDTMETHTFGVAPMGGENITIDGLQIGTDATADQDKPIYADKTFQPEPQVGEENWQETESFYGGRALKKDTSMKPCYGSYARPTNVKGGQAKLKVGADGVPTKEFDIDLAFFDTPGGTVNGQDEYKADIVMYTENTYLETPDTHVVYKPGKDDASSEINLVQQSMPNRPNYIGFRDNFIGLMYYNSTGNMGVLAGQASQLNAVVDLQDRNTELSYQLLLDSLGDRTRYFSMWNQAVDSYDPDVRIIENHGVEDELPNYCFPLDGSGTNAAYQGVKVKNGNDGDVESEWENDDTVAARNQLCKGNIFAMEINLQANLWRSFLYSNVALYLPDSYKYTPANITLPTNTNTYDYMNGRVVPPSLVDAYINIGARWSLDPMDNVNPFNHHRNAGLRYRSMLLGNGRYVPFHIQVPQKFFAIKSLLLLPGSYTYEWNFRKDVNMILQSSLGNDLRTDGASISFTSINLYATFFPMAHNTASTLEAMLRNDTNDQSFNDYLSAANMLYPIPANATNVPISIPSRNWAAFRGWSFTRLKTKETPSLGSGFDPYFVYSGSIPYLDGTFYLNHTFKKVSITFDSSVSWPGNDRLLTPNEFEIKRTVDGEGYNVAQCNMTKDWFLVQMLAHYNIGYQGFYVPEGYKDRMYSFFRNFQPMSRQVVDEVNYKDYQAVTLAYQHNNSGFVGYLAPTMRQGQPYPANYPYPLIGKSAVTSVTQKKFLCDRVMWRIPFSSNFMSMGALTDLGQNMLYANSAHALDMNFEVDPMDESTLLYVVFEVFDVVRVHQPHRGVIEAVYLRTPFSAGNATT

SEQ ID NO: 2 - protein, 942 aa, synthetic construct
MATPSMLPQWAYMHIAGQDASEYLSPGLVQFARATDTYFSLGNKFRNPTVAPTHDVTTDRSQRLTLRFVPVDREDNTYSYKVRYTLAVGDNRVLDMASTYFDIRGVLDRGPSFKPYSGTAYNSLAPKGAPNSSQWEQKKAGNGDTMETHTFGVAPMGGENITIDGLQIGTNATANQDKPIYADKTFQPEPQVGEENWQETESFYGGRALKKDTSMKPCYGSYARPTNVKGGQAKLKVGADGVPTKEFDIDLAFFDTPGGTVNGQDEYKADIVMYTENTYLETPDTHVVYKPGKDDASSEINLVQQSMPNRPNYIGFRDNFIGLMYYNSTGNMGVLAGQASQLNAVVDLQDRNTELSYQLLLDSLGDRTRYFSMWNQAVDSYDPDVRIIENHGVEDELPNYCFPLDGSGTNAAYQGVKVKNGNDGDVESEWENDDTVAARNQLCKGNIFAMEINLQANLWRSFLYSNVALYLPDSYKYTPANITLPTNTNTYDYMNGRVVPPSLVDAYINIGARWSLDPMDNVNPFNHHRNAGLRYRSMLLGNGRYVPFHIQVPQKFFAIKSLLLLPGSYTYEWNFRKDVNMILQSSLGNDLRTDGASISFTSINLYATFFPMAHNTASTLEAMLRNDTNDQSFNDYLSAANMLYPIPANATNVPISIPSRNWAAFRGWSFTRLKTKETPSLGSGFDPYFVYSGSIPYLDGTFYLNHTFKKVSITFDSSVSWPGNDRLLTPNEFEIKRTVDGEGYNVAQCNMTKDWFLVQMLAHYNIGYQGFYVPEGYKDRMYSFFRNFQPMSRQVVDEVNYKDYQAVTLAYQHNNSGFVGYLAPTMRQGQPYPANYPYPLIGKSAVTSVTQKKFLCDRVMWRIPFSSNFMSMGALTDLGQNMLYANSAHALDMNFEVDPMDESTLLYVVFEVFDVVRVHQPHRGVIEAVYLRTPFSAGNATT

SEQ ID NO: 3 - protein, 942 aa, synthetic construct
MATPSMLPQWAYMHIAGQDASEYLSPGLVQFARATDTYFSLGNKFRNPTVAPTHDVTTDRSQRLTLRFVPVDREDNTYSYKVRYTLAVGDNRVLDMASTYFDIRGVLDRGPSFKPYSGTAYNSLAPKGAPNSSQWEQKKAGNGDTMETHTFGVAPMGGENITIDGLQIGTDATANQNKPIYADKTFQPEPQVGEENWQETESFYGGRALKKDTSMKPCYGSYARPTNVKGGQAKLKVGADGVPTKEFDIDLAFFDTPGGTVNGQDEYKADIVMYTENTYLETPDTHVVYKPGKDDASSEINLVQQSMPNRPNYIGFRDNFIGLMYYNSTGNMGVLAGQASQLNAVVDLQDRNTELSYQLLLDSLGDRTRYFSMWNQAVDSYDPDVRIIENHGVEDELPNYCFPLDGSGTNAAYQGVKVKNGNDGDVESEWENDDTVAARNQLCKGNIFAMEINLQANLWRSFLYSNVALYLPDSYKYTPANITLPTNTNTYDYMNGRVVPPSLVDAYINIGARWSLDPMDNVNPFNHHRNAGLRYRSMLLGNGRYVPFHIQVPQKFFAIKSLLLLPGSYTYEWNFRKDVNMILQSSLGNDLRTDGASISFTSINLYATFFPMAHNTASTLEAMLRNDTNDQSFNDYLSAANMLYPIPANATNVPISIPSRNWAAFRGWSFTRLKTKETPSLGSGFDPYFVYSGSIPYLDGTFYLNHTFKKVSITFDSSVSWPGNDRLLTPNEFEIKRTVDGEGYNVAQCNMTKDWFLVQMLAHYNIGYQGFYVPEGYKDRMYSFFRNFQPMSRQVVDEVNYKDYQAVTLAYQHNNSGFVGYLAPTMRQGQPYPANYPYPLIGKSAVTSVTQKKFLCDRVMWRIPFSSNFMSMGALTDLGQNMLYANSAHALDMNFEVDPMDESTLLYVVFEVFDVVRVHQPHRGVIEAVYLRTPFSAGNATT

SEQ ID NO: 4 - protein, 942 aa, synthetic construct
MATPSMLPQWAYMHIAGQDASEYLSPGLVQFARATDTYFSLGNKFRNPTVAPTHDVTTDRSQRLTLRFVPVDREDNTYSYKVRYTLAVGDNRVLDMASTYFDIRGVLDRGPSFKPYSGTAYNSLAPKGAPNSSQWEQKKAGNGDTMETHTFGVAPMGGENITIDGLQIGTNATADQNKPIYADKTFQPEPQVGEENWQETESFYGGRALKKDTSMKPCYGSYARPTNVKGGQAKLKVGADGVPTKEFDIDLAFFDTPGGTVNGQDEYKADIVMYTENTYLETPDTHVVYKPGKDDASSEINLVQQSMPNRPNYIGFRDNFIGLMYYNSTGNMGVLAGQASQLNAVVDLQDRNTELSYQLLLDSLGDRTRYFSMWNQAVDSYDPDVRIIENHGVEDELPNYCFPLDGSGTNAAYQGVKVKNGNDGDVESEWENDDTVAARNQLCKGNIFAMEINLQANLWRSFLYSNVALYLPDSYKYTPANITLPTNTNTYDYMNGRVVPPSLVDAYINIGARWSLDPMDNVNPFNHHRNAGLRYRSMLLGNGRYVPFHIQVPQKFFAIKSLLLLPGSYTYEWNFRKDVNMILQSSLGNDLRTDGASISFTSINLYATFFPMAHNTASTLEAMLRNDTNDQSFNDYLSAANMLYPIPANATNVPISIPSRNWAAFRGWSFTRLKTKETPSLGSGFDPYFVYSGSIPYLDGTFYLNHTFKKVSITFDSSVSWPGNDRLLTPNEFEIKRTVDGEGYNVAQCNMTKDWFLVQMLAHYNIGYQGFYVPEGYKDRMYSFFRNFQPMSRQVVDEVNYKDYQAVTLAYQHNNSGFVGYLAPTMRQGQPYPANYPYPLIGKSAVTSVTQKKFLCDRVMWRIPFSSNFMSMGALTDLGQNMLYANSAHALDMNFEVDPMDESTLLYVVFEVFDVVRVHQPHRGVIEAVYLRTPFSAGNATT

SEQ ID NO: 5 - protein, 942 aa, synthetic construct
MATPSMLPQWAYMHIAGQDASEYLSPGLVQFARATDTYFSLGNKFRNPTVAPTHDVTTDRSQRLTLRFVPVDREDNTYSYKVRYTLAVGDNRVLDMASTYFDIRGVLDRGPSFKPYSGTAYNSLAPKGAPNSSQWEQKKAGNGDTMETHTFGVAPMGGENITIDGLQIGTNATANQNKPIYADKTFQPEPQVGEENWQETESFYGGRALKKDTSMKPCYGSYARPTNVKGGQAKLKVGADGVPTKEFDIDLAFFDTPGGTVNGQDEYKADIVMYTENTYLETPDTHVVYKPGKDDASSEINLVQQSMPNRPNYIGFRDNFIGLMYYNSTGNMGVLAGQASQLNAVVDLQDRNTELSYQLLLDSLGDRTRYFSMWNQAVDSYDPDVRIIENHGVEDELPNYCFPLDGSGTNAAYQGVKVKNGNDGDVESEWENDDTVAARNQLCKGNIFAMEINLQANLWRSFLYSNVALYLPDSYKYTPANITLPTNTNTYDYMNGRVVPPSLVDAYINIGARWSLDPMDNVNPFNHHRNAGLRYRSMLLGNGRYVPFHIQVPQKFFAIKSLLLLPGSYTYEWNFRKDVNMILQSSLGNDLRTDGASISFTSINLYATFFPMAHNTASTLEAMLRNDTNDQSFNDYLSAANMLYPIPANATNVPISIPSRNWAAFRGWSFTRLKTKETPSLGSGFDPYFVYSGSIPYLDGTFYLNHTFKKVSITFDSSVSWPGNDRLLTPNEFEIKRTVDGEGYNVAQCNMTKDWFLVQMLAHYNIGYQGFYVPEGYKDRMYSFFRNFQPMSRQVVDEVNYKDYQAVTLAYQHNNSGFVGYLAPTMRQGQPYPANYPYPLIGKSAVTSVTQKKFLCDRVMWRIPFSSNFMSMGALTDLGQNMLYANSAHALDMNFEVDPMDESTLLYVVFEVFDVVRVHQPHRGVIEAVYLRTPFSAGNATT

SEQ ID NO: 6 - protein, 942 aa, synthetic construct
MATPSMLPQWAYMHIAGQDASEYLSPGLVQFARATDTYFSLGNKFRNPTVAPTHDVTTDRSQRLTLRFVPVDREDNTYSYKVRYTLAVGDNRVLDMASTYFDIRGVLDRGPSFKPYSGTAYNSLAPKGAPNSSQWEQKKAGNGDTMETHTFGVAPMGGENITIDGLQIGTDATANQNKPIYANKTFQPEPQVGEENWQETESFYGGRALKKDTSMKPCYGSYARPTNVKGGQAKLKVGADGVPTKEFDIDLAFFDTPGGTVNGQDEYKADIVMYTENTYLETPDTHVVYKPGKDDASSEINLVQQSMPNRPNYIGFRDNFIGLMYYNSTGNMGVLAGQASQLNAVVDLQDRNTELSYQLLLDSLGDRTRYFSMWNQAVDSYDPDVRIIENHGVEDELPNYCFPLDGSGTNAAYQGVKVKNGNDGDVESEWENDDTVAARNQLCKGNIFAMEINLQANLWRSFLYSNVALYLPDSYKYTPANITLPTNTNTYDYMNGRVVPPSLVDAYINIGARWSLDPMDNVNPFNHHRNAGLRYRSMLLGNGRYVPFHIQVPQKFFAIKSLLLLPGSYTYEWNFRKDVNMILQSSLGNDLRTDGASISFTSINLYATFFPMAHNTASTLEAMLRNDTNDQSFNDYLSAANMLYPIPANATNVPISIPSRNWAAFRGWSFTRLKTKETPSLGSGFDPYFVYSGSIPYLDGTFYLNHTFKKVSITFDSSVSWPGNDRLLTPNEFEIKRTVDGEGYNVAQCNMTKDWFLVQMLAHYNIGYQGFYVPEGYKDRMYSFFRNFQPMSRQVVDEVNYKDYQAVTLAYQHNNSGFVGYLAPTMRQGQPYPANYPYPLIGKSAVTSVTQKKFLCDRVMWRIPFSSNFMSMGALTDLGQNMLYANSAHALDMNFEVDPMDESTLLYVVFEVFDVVRVHQPHRGVIEAVYLRTPFSAGNATT

SEQ ID NO: 7 - protein, 942 aa, synthetic construct
MATPSMLPQWAYMHIAGQDASEYLSPGLVQFARATDTYFSLGNKFRNPTVAPTHDVTTDRSQRLTLRFVPVDREDNTYSYKVRYTLAVGDNRVLDMASTYFDIRGVLDRGPSFKPYSGTAYNSLAPKGAPNSSQWEQKKAGNGDTMETHTFGVAPMGGENITIDGLQIGTNATADQNKPIYANKTFQPEPQVGEENWQETESFYGGRALKKDTSMKPCYGSYARPTNVKGGQAKLKVGADGVPTKEFDIDLAFFDTPGGTVNGQDEYKADIVMYTENTYLETPDTHVVYKPGKDDASSEINLVQQSMPNRPNYIGFRDNFIGLMYYNSTGNMGVLAGQASQLNAVVDLQDRNTELSYQLLLDSLGDRTRYFSMWNQAVDSYDPDVRIIENHGVEDELPNYCFPLDGSGTNAAYQGVKVKNGNDGDVESEWENDDTVAARNQLCKGNIFAMEINLQANLWRSFLYSNVALYLPDSYKYTPANITLPTNTNTYDYMNGRVVPPSLVDAYINIGARWSLDPMDNVNPFNHHRNAGLRYRSMLLGNGRYVPFHIQVPQKFFAIKSLLLLPGSYTYEWNFRKDVNMILQSSLGNDLRTDGASISFTSINLYATFFPMAHNTASTLEAMLRNDTNDQSFNDYLSAANMLYPIPANATNVPISIPSRNWAAFRGWSFTRLKTKETPSLGSGFDPYFVYSGSIPYLDGTFYLNHTFKKVSITFDSSVSWPGNDRLLTPNEFEIKRTVDGEGYNVAQCNMTKDWFLVQMLAHYNIGYQGFYVPEGYKDRMYSFFRNFQPMSRQVVDEVNYKDYQAVTLAYQHNNSGFVGYLAPTMRQGQPYPANYPYPLIGKSAVTSVTQKKFLCDRVMWRIPFSSNFMSMGALTDLGQNMLYANSAHALDMNFEVDPMDESTLLYVVFEVFDVVRVHQPHRGVIEAVYLRTPFSAGNATT

SEQ ID NO: 8 - protein, 942 aa, synthetic construct
MATPSMLPQWAYMHIAGQDASEYLSPGLVQFARATDTYFSLGNKFRNPTVAPTHDVTTDRSQRLTLRFVPVDREDNTYSYKVRYTLAVGDNRVLDMASTYFDIRGVLDRGPSFKPYSGTAYNSLAPKGAPNSSQWEQKKAGNGDTMETHTFGVAPMGGENITIDGLQIGTDATADQDKPIYADKTFQPEPQVGEENWQETESFYGGRALKKDTSMKPCYGSYARPTNVKGGQAKLKVGADGVPTKEFDIDLAFFDTPGGTVNGQDEYKADIVMYTENTYLETPDTHVVYKPGKDDASSEINLVQQSMPNRPNYIGFRDNFIGLMYYNSTGNMGVLAGQASQLNAVVDLQDRNTELSYQLLLDSLGDRTRYFSMWNQAVDSYDPDVRIIENHGVEDELPNYCFPLDGSGTNAAYQGVKVKNGNNGNVQSQWENNNTVAARNQLCKGNIFAMEINLQANLWRSFLYSNVALYLPDSYKYTPANITLPTNTNTYDYMNGRVVPPSLVDAYINIGARWSLDPMDNVNPFNHHRNAGLRYRSMLLGNGRYVPFHIQVPQKFFAIKSLLLLPGSYTYEWNFRKDVNMILQSSLGNDLRTDGASISFTSINLYATFFPMAHNTASTLEAMLRNDTNDQSFNDYLSAANMLYPIPANATNVPISIPSRNWAAFRGWSFTRLKTKETPSLGSGFDPYFVYSGSIPYLDGTFYLNHTFKKVSITFDSSVSWPGNDRLLTPNEFEIKRTVDGEGYNVAQCNMTKDWFLVQMLAHYNIGYQGFYVPEGYKDRMYSFFRNFQPMSRQVVDEVNYKDYQAVTLAYQHNNSGFVGYLAPTMRQGQPYPANYPYPLIGKSAVTSVTQKKFLCDRVMWRIPFSSNFMSMGALTDLGQNMLYANSAHALDMNFEVDPMDESTLLYVVFEVFDVVRVHQPHRGVIEAVYLRTPFSAGNATT

SEQ ID NO: 9 - protein, 942 aa, synthetic construct
MATPSMLPQWAYMHIAGQDASEYLSPGLVQFARATDTYFSLGNKFRNPTVAPTHDVTTDRSQRLTLRFVPVDREDNTYSYKVRYTLAVGDNRVLDMASTYFDIRGVLDRGPSFKPYSGTAYNSLAPKGAPNSSQWEQKKAGNGDTMETHTFGVAPMGGENITIDGLQIGTDATADQDKPIYADKTFQPEPQVGEENWQETESFYGGRALKKDTSMKPCYGSYARPTNVKGGQAKLKVGADGVPTKEFDIDLAFFDTPGGTVNGQDEYKADIVMYTENTYLETPDTHVVYKPGKDDASSEINLVQQSMPNRPNYIGFRDNFIGLMYYNSTGNMGVLAGQASQLNAVVDLQDRNTELSYQLLLDSLGDRTRYFSMWNQAVDSYDPDVRIIENHGVEDELPNYCFPLDGSGTNAAYQGVKVKNGNNGNVQSQWENDDTVAARNQLCKGNIFAMEINLQANLWRSFLYSNVALYLPDSYKYTPANITLPTNTNTYDYMNGRVVPPSLVDAYINIGARWSLDPMDNVNPFNHHRNAGLRYRSMLLGNGRYVPFHIQVPQKFFAIKSLLLLPGSYTYEWNFRKDVNMILQSSLGNDLRTDGASISFTSINLYATFFPMAHNTASTLEAMLRNDTNDQSFNDYLSAANMLYPIPANATNVPISIPSRNWAAFRGWSFTRLKTKETPSLGSGFDPYFVYSGSIPYLDGTFYLNHTFKKVSITFDSSVSWPGNDRLLTPNEFEIKRTVDGEGYNVAQCNMTKDWFLVQMLAHYNIGYQGFYVPEGYKDRMYSFFRNFQPMSRQVVDEVNYKDYQAVTLAYQHNNSGFVGYLAPTMRQGQPYPANYPYPLIGKSAVTSVTQKKFLCDRVMWRIPFSSNFMSMGALTDLGQNMLYANSAHALDMNFEVDPMDESTLLYVVFEVFDVVRVHQPHRGVIEAVYLRTPFSAGNATT

SEQ ID NO: 10 - protein, 942 aa, synthetic construct
MATPSMLPQWAYMHIAGQDASEYLSPGLVQFARATDTYFSLGNKFRNPTVAPTHDVTTDRSQRLTLRFVPVDREDNTYSYKVRYTLAVGDNRVLDMASTYFDIRGVLDRGPSFKPYSGTAYNSLAPKGAPNSSQWEQKKAGNGDTMETHTFGVAPMGGENITIDGLQIGTDATADQDKPIYADKTFQPEPQVGEENWQETESFYGGRALKKDTSMKPCYGSYARPTNVKGGQAKLKVGADGVPTKEFDIDLAFFDTPGGTVNGQDEYKADIVMYTENTYLETPDTHVVYKPGKDDASSEINLVQQSMPNRPNYIGFRDNFIGLMYYNSTGNMGVLAGQASQLNAVVDLQDRNTELSYQLLLDSLGDRTRYFSMWNQAVDSYDPDVRIIENHGVEDELPNYCFPLDGSGTNAAYQGVKVKNGNNGNVESEWENNNTVAARNQLCKGNIFAMEINLQANLWRSFLYSNVALYLPDSYKYTPANITLPTNTNTYDYMNGRVVPPSLVDAYINIGARWSLDPMDNVNPFNHHRNAGLRYRSMLLGNGRYVPFHIQVPQKFFAIKSLLLLPGSYTYEWNFRKDVNMILQSSLGNDLRTDGASISFTSINLYATFFPMAHNTASTLEAMLRNDTNDQSFNDYLSAANMLYPIPANATNVPISIPSRNWAAFRGWSFTRLKTKETPSLGSGFDPYFVYSGSIPYLDGTFYLNHTFKKVSITFDSSVSWPGNDRLLTPNEFEIKRTVDGEGYNVAQCNMTKDWFLVQMLAHYNIGYQGFYVPEGYKDRMYSFFRNFQPMSRQVVDEVNYKDYQAVTLAYQHNNSGFVGYLAPTMRQGQPYPANYPYPLIGKSAVTSVTQKKFLCDRVMWRIPFSSNFMSMGALTDLGQNMLYANSAHALDMNFEVDPMDESTLLYVVFEVFDVVRVHQPHRGVIEAVYLRTPFSAGNATT

SEQ ID NO: 11 - protein, 942 aa, synthetic construct
MATPSMLPQWAYMHIAGQDASEYLSPGLVQFARATDTYFSLGNKFRNPTVAPTHDVTTDRSQRLTLRFVPVDREDNTYSYKVRYTLAVGDNRVLDMASTYFDIRGVLDRGPSFKPYSGTAYNSLAPKGAPNSSQWEQKKAGNGDTMETHTFGVAPMGGENITIDGLQIGTDATADQDKPIYADKTFQPEPQVGEENWQETESFYGGRALKKDTSMKPCYGSYARPTNVKGGQAKLKVGADGVPTKEFDIDLAFFDTPGGTVNGQDEYKADIVMYTENTYLETPDTHVVYKPGKDDASSEINLVQQSMPNRPNYIGFRDNFIGLMYYNSTGNMGVLAGQASQLNAVVDLQDRNTELSYQLLLDSLGDRTRYFSMWNQAVDSYDPDVRIIENHGVEDELPNYCFPLDGSGTNAAYQGVKVKNGNDGDVESEWENNNTVAARNQLCKGNIFAMEINLQANLWRSFLYSNVALYLPDSYKYTPANITLPTNTNTYDYMNGRVVPPSLVDAYINIGARWSLDPMDNVNPFNHHRNAGLRYRSMLLGNGRYVPFHIQVPQKFFAIKSLLLLPGSYTYEWNFRKDVNMILQSSLGNDLRTDGASISFTSINLYATFFPMAHNTASTLEAMLRNDTNDQSFNDYLSAANMLYPIPANATNVPISIPSRNWAAFRGWSFTRLKTKETPSLGSGFDPYFVYSGSIPYLDGTFYLNHTFKKVSITFDSSVSWPGNDRLLTPNEFEIKRTVDGEGYNVAQCNMTKDWFLVQMLAHYNIGYQGFYVPEGYKDRMYSFFRNFQPMSRQVVDEVNYKDYQAVTLAYQHNNSGFVGYLAPTMRQGQPYPANYPYPLIGKSAVTSVTQKKFLCDRVMWRIPFSSNFMSMGALTDLGQNMLYANSAHALDMNFEVDPMDESTLLYVVFEVFDVVRVHQPHRGVIEAVYLRTPFSAGNATT

SEQ ID NO: 12 - protein, 942 aa, synthetic construct
MATPSMLPQWAYMHIAGQDASEYLSPGLVQFARATDTYFSLGNKFRNPTVAPTHDVTTDRSQRLTLRFVPVDREDNTYSYKVRYTLAVGDNRVLDMASTYFDIRGVLDRGPSFKPYSGTAYNSLAPKGAPNSSQWEQKKAGNGDTMETHTFGVAPMGGENITIDGLQIGTDATADQDKPIYADKTFQPEPQVGEENWQETESFYGGRALKKDTSMKPCYGSYARPTNVKGGQAKLKVGADGVPTKEFDIDLAFFDTPGGTVNGQDEYKADIVMYTENTYLETPDTHVVYKPGKDDASSEINLVQQSMPNRPNYIGFRDNFIGLMYYNSTGNMGVLAGQASQLNAVVDLQDRNTELSYQLLLDSLGDRTRYFSMWNQAVDSYDPDVRIIENHGVEDELPNYCFPLDGSGTNAAYQGVKVKNGNNGNVESEWENNDTVAARNQLCKGNIFAMEINLQANLWRSFLYSNVALYLPDSYKYTPANITLPTNTNTYDYMNGRVVPPSLVDAYINIGARWSLDPMDNVNPFNHHRNAGLRYRSMLLGNGRYVPFHIQVPQKFFAIKSLLLLPGSYTYEWNFRKDVNMILQSSLGNDLRTDGASISFTSINLYATFFPMAHNTASTLEAMLRNDTNDQSFNDYLSAANMLYPIPANATNVPISIPSRNWAAFRGWSFTRLKTKETPSLGSGFDPYFVYSGSIPYLDGTFYLNHTFKKVSITFDSSVSWPGNDRLLTPNEFEIKRTVDGEGYNVAQCNMTKDWFLVQMLAHYNIGYQGFYVPEGYKDRMYSFFRNFQPMSRQVVDEVNYKDYQAVTLAYQHNNSGFVGYLAPTMRQGQPYPANYPYPLIGKSAVTSVTQKKFLCDRVMWRIPFSSNFMSMGALTDLGQNMLYANSAHALDMNFEVDPMDESTLLYVVFEVFDVVRVHQPHRGVIEAVYLRTPFSAGNATT

SEQ ID NO: 13 - protein, 942 aa, synthetic construct
MATPSMLPQWAYMHIAGQDASEYLSPGLVQFARATDTYFSLGNKFRNPTVAPTHDVTTDRSQRLTLRFVPVDREDNTYSYKVRYTLAVGDNRVLDMASTYFDIRGVLDRGPSFKPYSGTAYNSLAPKGAPNSSQWEQKKAGNGDTMETHTFGVAPMGGENITIDGLQIGTDATADQDKPIYADKTFQPEPQVGEENWQETESFYGGRALKKDTSMKPCYGSYARPTNVKGGQAKLKVGADGVPTKEFDIDLAFFDTPGGTVNGQDEYKADIVMYTENTYLETPDTHVVYKPGKDDASSEINLVQQSMPNRPNYIGFRDNFIGLMYYNSTGNMGVLAGQASQLNAVVDLQDRNTELSYQLLLDSLGDRTRYFSMWNQAVDSYDPDVRIIENHGVEDELPNYCFPLDGSGTNAAYQGVKVKNGNNGNVQSEWENDDTVAARNQLCKGNIFAMEINLQANLWRSFLYSNVALYLPDSYKYTPANITLPTNTNTYDYMNGRVVPPSLVDAYINIGARWSLDPMDNVNPFNHHRNAGLRYRSMLLGNGRYVPFHIQVPQKFFAIKSLLLLPGSYTYEWNFRKDVNMILQSSLGNDLRTDGASISFTSINLYATFFPMAHNTASTLEAMLRNDTNDQSFNDYLSAANMLYPIPANATNVPISIPSRNWAAFRGWSFTRLKTKETPSLGSGFDPYFVYSGSIPYLDGTFYLNHTFKKVSITFDSSVSWPGNDRLLTPNEFEIKRTVDGEGYNVAQCNMTKDWFLVQMLAHYNIGYQGFYVPEGYKDRMYSFFRNFQPMSRQVVDEVNYKDYQAVTLAYQHNNSGFVGYLAPTMRQGQPYPANYPYPLIGKSAVTSVTQKKFLCDRVMWRIPFSSNFMSMGALTDLGQNMLYANSAHALDMNFEVDPMDESTLLYVVFEVFDVVRVHQPHRGVIEAVYLRTPFSAGNATT

SEQ ID NO: 14 - protein, 942 aa, synthetic construct
MATPSMLPQWAYMHIAGQDASEYLSPGLVQFARATDTYFSLGNKFRNPTVAPTHDVTTDRSQRLTLRFVPVDREDNTYSYKVRYTLAVGDNRVLDMASTYFDIRGVLDRGPSFKPYSGTAYNSLAPKGAPNSSQWEQKKAGNGDTMETHTFGVAPMGGENITIDGLQIGTDATADQDKPIYADKTFQPEPQVGEENWQETESFYGGRALKKDTSMKPCYGSYARPTNVKGGQAKLKVGADGVPTKEFDIDLAFFDTPGGTVNGQDEYKADIVMYTENTYLETPDTHVVYKPGKDDASSEINLVQQSMPNRPNYIGFRDNFIGLMYYNSTGNMGVLAGQASQLNAVVDLQDRNTELSYQLLLDSLGDRTRYFSMWNQAVDSYDPDVRIIENHGVEDELPNYCFPLDGSGTNAAYQGVKVKNGNNGNVQSQWENNDTVAARNQLCKGNIFAMEINLQANLWRSFLYSNVALYLPDSYKYTPANITLPTNTNTYDYMNGRVVPPSLVDAYINIGARWSLDPMDNVNPFNHHRNAGLRYRSMLLGNGRYVPFHIQVPQKFFAIKSLLLLPGSYTYEWNFRKDVNMILQSSLGNDLRTDGASISFTSINLYATFFPMAHNTASTLEAMLRNDTNDQSFNDYLSAANMLYPIPANATNVPISIPSRNWAAFRGWSFTRLKTKETPSLGSGFDPYFVYSGSIPYLDGTFYLNHTFKKVSITFDSSVSWPGNDRLLTPNEFEIKRTVDGEGYNVAQCNMTKDWFLVQMLAHYNIGYQGFYVPEGYKDRMYSFFRNFQPMSRQVVDEVNYKDYQAVTLAYQHNNSGFVGYLAPTMRQGQPYPANYPYPLIGKSAVTSVTQKKFLCDRVMWRIPFSSNFMSMGALTDLGQNMLYANSAHALDMNFEVDPMDESTLLYVVFEVFDVVRVHQPHRGVIEAVYLRTPFSAGNATT

SEQ ID NO: 15 - protein, 942 aa, synthetic construct
MATPSMLPQWAYMHIAGQDASEYLSPGLVQFARATDTYFSLGNKFRNPTVAPTHDVTTDRSQRLTLRFVPVDREDNTYSYKVRYTLAVGDNRVLDMASTYFDIRGVLDRGPSFKPYSGTAYNSLAPKGAPNSSQWEQKKAGNGDTMETHTFGVAPMGGENITIDGLQIGTDATADQDKPIYADKTFQPEPQVGEENWQETESFYGGRALKKDTSMKPCYGSYARPTNVKGGQAKLKVGADGVPTKEFDIDLAFFDTPGGTVNGQDEYKADIVMYTENTYLETPDTHVVYKPGKDDASSEINLVQQSMPNRPNYIGFRDNFIGLMYYNSTGNMGVLAGQASQLNAVVDLQDRNTELSYQLLLDSLGDRTRYFSMWNQAVDSYDPDVRIIENHGVEDELPNYCFPLDGSGTNAAYQGVKVKNGNNGNVQSQWENDNTVAARNQLCKGNIFAMEINLQANLWRSFLYSNVALYLPDSYKYTPANITLPTNTNTYDYMNGRVVPPSLVDAYINIGARWSLDPMDNVNPFNHHRNAGLRYRSMLLGNGRYVPFHIQVPQKFFAIKSLLLLPGSYTYEWNFRKDVNMILQSSLGNDLRTDGASISFTSINLYATFFPMAHNTASTLEAMLRNDTNDQSFNDYLSAANMLYPIPANATNVPISIPSRNWAAFRGWSFTRLKTKETPSLGSGFDPYFVYSGSIPYLDGTFYLNHTFKKVSITFDSSVSWPGNDRLLTPNEFEIKRTVDGEGYNVAQCNMTKDWFLVQMLAHYNIGYQGFYVPEGYKDRMYSFFRNFQPMSRQVVDEVNYKDYQAVTLAYQHNNSGFVGYLAPTMRQGQPYPANYPYPLIGKSAVTSVTQKKFLCDRVMWRIPFSSNFMSMGALTDLGQNMLYANSAHALDMNFEVDPMDESTLLYVVFEVFDVVRVHQPHRGVIEAVYLRTPFSAGNATT

SEQ ID NO: 16 - protein, 942 aa, synthetic construct
MATPSMLPQWAYMHIAGQDASEYLSPGLVQFARATDTYFSLGNKFRNPTVAPTHDVTTDRSQRLTLRFVPVDREDNTYSYKVRYTLAVGDNRVLDMASTYFDIRGVLDRGPSFKPYSGTAYNSLAPKGAPNSSQWEQKKAGNGDTMETHTFGVAPMGGENITIDGLQIGTNATANQNKPIYADKTFQPEPQVGEENWQETESFYGGRALKKDTSMKPCYGSYARPTNVKGGQAKLKVGADGVPTKEFDIDLAFFDTPGGTVNGQDEYKADIVMYTENTYLETPDTHVVYKPGKDDASSEINLVQQSMPNRPNYIGFRDNFIGLMYYNSTGNMGVLAGQASQLNAVVDLQDRNTELSYQLLLDSLGDRTRYFSMWNQAVDSYDPDVRIIENHGVEDELPNYCFPLDGSGTNAAYQGVKVKNGNNGNVQSQWENDDTVAARNQLCKGNIFAMEINLQANLWRSFLYSNVALYLPDSYKYTPANITLPTNTNTYDYMNGRVVPPSLVDAYINIGARWSLDPMDNVNPFNHHRNAGLRYRSMLLGNGRYVPFHIQVPQKFFAIKSLLLLPGSYTYEWNFRKDVNMILQSSLGNDLRTDGASISFTSINLYATFFPMAHNTASTLEAMLRNDTNDQSFNDYLSAANMLYPIPANATNVPISIPSRNWAAFRGWSFTRLKTKETPSLGSGFDPYFVYSGSIPYLDGTFYLNHTFKKVSITFDSSVSWPGNDRLLTPNEFEIKRTVDGEGYNVAQCNMTKDWFLVQMLAHYNIGYQGFYVPEGYKDRMYSFFRNFQPMSRQVVDEVNYKDYQAVTLAYQHNNSGFVGYLAPTMRQGQPYPANYPYPLIGKSAVTSVTQKKFLCDRVMWRIPFSSNFMSMGALTDLGQNMLYANSAHALDMNFEVDPMDESTLLYVVFEVFDVVRVHQPHRGVIEAVYLRTPFSAGNATT

SEQ ID NO: 17 - protein, 942 aa, synthetic construct
MATPSMLPQWAYMHIAGQDASEYLSPGLVQFARATDTYFSLGNKFRNPTVAPTHDVTTDRSQRLTLRFVPVDREDNTYSYKVRYTLAVGDNRVLDMASTYFDIRGVLDRGPSFKPYSGTAYNSLAPKGAPNSSQWEQKKAGNGDTMETHTFGVAPMGGENITIDGLQIGTKATAKQKKPIYADKTFQPEPQVGEENWQETESFYGGRALKKDTSMKPCYGSYARPTNVKGGQAKLKVGADGVPTKEFDIDLAFFDTPGGTVNGQDEYKADIVMYTENTYLETPDTHVVYKPGKDDASSEINLVQQSMPNRPNYIGFRDNFIGLMYYNSTGNMGVLAGQASQLNAVVDLQDRNTELSYQLLLDSLGDRTRYFSMWNQAVDSYDPDVRIIENHGVEDELPNYCFPLDGSGTNAAYQGVKVKNGNKGKVKSKWENDDTVAARNQLCKGNIFAMEINLQANLWRSFLYSNVALYLPDSYKYTPANITLPTNTNTYDYMNGRVVPPSLVDAYINIGARWSLDPMDNVNPFNHHRNAGLRYRSMLLGNGRYVPFHIQVPQKFFAIKSLLLLPGSYTYEWNFRKDVNMILQSSLGNDLRTDGASISFTSINLYATFFPMAHNTASTLEAMLRNDTNDQSFNDYLSAANMLYPIPANATNVPISIPSRNWAAFRGWSFTRLKTKETPSLGSGFDPYFVYSGSIPYLDGTFYLNHTFKKVSITFDSSVSWPGNDRLLTPNEFEIKRTVDGEGYNVAQCNMTKDWFLVQMLAHYNIGYQGFYVPEGYKDRMYSFFRNFQPMSRQVVDEVNYKDYQAVTLAYQHNNSGFVGYLAPTMRQGQPYPANYPYPLIGKSAVTSVTQKKFLCDRVMWRIPFSSNFMSMGALTDLGQNMLYANSAHALDMNFEVDPMDESTLLYVVFEVFDVVRVHQPHRGVIEAVYLRTPFSAGNATT

SEQ ID NO: 18 - protein, 942 aa, synthetic construct
MATPSMLPQWAYMHIAGQDASEYLSPGLVQFARATDTYFSLGNKFRNPTVAPTHDVTTDRSQRLTLRFVPVDREDNTYSYKVRYTLAVGDNRVLDMASTYFDIRGVLDRGPSFKPYSGTAYNSLAPKGAPNSSQWEQKKAGNGDTMETHTFGVAPMGGENITIDGLQIGTKATANQNKPIYADKTFQPEPQVGEENWQETESFYGGRALKKDTSMKPCYGSYARPTNVKGGQAKLKVGADGVPTKEFDIDLAFFDTPGGTVNGQDEYKADIVMYTENTYLETPDTHVVYKPGKDDASSEINLVQQSMPNRPNYIGFRDNFIGLMYYNSTGNMGVLAGQASQLNAVVDLQDRNTELSYQLLLDSLGDRTRYFSMWNQAVDSYDPDVRIIENHGVEDELPNYCFPLDGSGTNAAYQGVKVKNGNNGNVQSQWENDDTVAARNQLCKGNIFAMEINLQANLWRSFLYSNVALYLPDSYKYTPANITLPTNTNTYDYMNGRVVPPSLVDAYINIGARWSLDPMDNVNPFNHHRNAGLRYRSMLLGNGRYVPFHIQVPQKFFAIKSLLLLPGSYTYEWNFRKDVNMILQSSLGNDLRTDGASISFTSINLYATFFPMAHNTASTLEAMLRNDTNDQSFNDYLSAANMLYPIPANATNVPISIPSRNWAAFRGWSFTRLKTKETPSLGSGFDPYFVYSGSIPYLDGTFYLNHTFKKVSITFDSSVSWPGNDRLLTPNEFEIKRTVDGEGYNVAQCNMTKDWFLVQMLAHYNIGYQGFYVPEGYKDRMYSFFRNFQPMSRQVVDEVNYKDYQAVTLAYQHNNSGFVGYLAPTMRQGQPYPANYPYPLIGKSAVTSVTQKKFLCDRVMWRIPFSSNFMSMGALTDLGQNMLYANSAHALDMNFEVDPMDESTLLYVVFEVFDVVRVHQPHRGVIEAVYLRTPFSAGNATT

SEQ ID NO: 19 - protein, 942 aa, synthetic construct
MATPSMLPQWAYMHIAGQDASEYLSPGLVQFARATDTYFSLGNKFRNPTVAPTHDVTTDRSQRLTLRFVPVDREDNTYSYKVRYTLAVGDNRVLDMASTYFDIRGVLDRGPSFKPYSGTAYNSLAPKGAPNSSQWEQKKAGNGDTMETHTFGVAPMGGENITIDGLQIGTKATAKQNKPIYADKTFQPEPQVGEENWQETESFYGGRALKKDTSMKPCYGSYARPTNVKGGQAKLKVGADGVPTKEFDIDLAFFDTPGGTVNGQDEYKADIVMYTENTYLETPDTHVVYKPGKDDASSEINLVQQSMPNRPNYIGFRDNFIGLMYYNSTGNMGVLAGQASQLNAVVDLQDRNTELSYQLLLDSLGDRTRYFSMWNQAVDSYDPDVRIIENHGVEDELPNYCFPLDGSGTNAAYQGVKVKNGNNGNVQSQWENDDTVAARNQLCKGNIFAMEINLQANLWRSFLYSNVALYLPDSYKYTPANITLPTNTNTYDYMNGRVVPPSLVDAYINIGARWSLDPMDNVNPFNHHRNAGLRYRSMLLGNGRYVPFHIQVPQKFFAIKSLLLLPGSYTYEWNFRKDVNMILQSSLGNDLRTDGASISFTSINLYATFFPMAHNTASTLEAMLRNDTNDQSFNDYLSAANMLYPIPANATNVPISIPSRNWAAFRGWSFTRLKTKETPSLGSGFDPYFVYSGSIPYLDGTFYLNHTFKKVSITFDSSVSWPGNDRLLTPNEFEIKRTVDGEGYNVAQCNMTKDWFLVQMLAHYNIGYQGFYVPEGYKDRMYSFFRNFQPMSRQVVDEVNYKDYQAVTLAYQHNNSGFVGYLAPTMRQGQPYPANYPYPLIGKSAVTSVTQKKFLCDRVMWRIPFSSNFMSMGALTDLGQNMLYANSAHALDMNFEVDPMDESTLLYVVFEVFDVVRVHQPHRGVIEAVYLRTPFSAGNATT

SEQ ID NO: 20 - protein, 942 aa, synthetic construct
MATPSMLPQWAYMHIAGQDASEYLSPGLVQFARATDTYFSLGNKFRNPTVAPTHDVTTDRSQRLTLRFVPVDREDNTYSYKVRYTLAVGDNRVLDMASTYFDIRGVLDRGPSFKPYSGTAYNSLAPKGAPNSSQWEQKKAGNGDTMETHTFGVAPMGGENITIDGLQIGTKATAKQKKPIYADKTFQPEPQVGEENWQETESFYGGRALKKDTSMKPCYGSYARPTNVKGGQAKLKVGADGVPTKEFDIDLAFFDTPGGTVNGQDEYKADIVMYTENTYLETPDTHVVYKPGKDDASSEINLVQQSMPNRPNYIGFRDNFIGLMYYNSTGNMGVLAGQASQLNAVVDLQDRNTELSYQLLLDSLGDRTRYFSMWNQAVDSYDPDVRIIENHGVEDELPNYCFPLDGSGTNAAYQGVKVKNGNNGNVQSQWENDDTVAARNQLCKGNIFAMEINLQANLWRSFLYSNVALYLPDSYKYTPANITLPTNTNTYDYMNGRVVPPSLVDAYINIGARWSLDPMDNVNPFNHHRNAGLRYRSMLLGNGRYVPFHIQVPQKFFAIKSLLLLPGSYTYEWNFRKDVNMILQSSLGNDLRTDGASISFTSINLYATFFPMAHNTASTLEAMLRNDTNDQSFNDYLSAANMLYPIPANATNVPISIPSRNWAAFRGWSFTRLKTKETPSLGSGFDPYFVYSGSIPYLDGTFYLNHTFKKVSITFDSSVSWPGNDRLLTPNEFEIKRTVDGEGYNVAQCNMTKDWFLVQMLAHYNIGYQGFYVPEGYKDRMYSFFRNFQPMSRQVVDEVNYKDYQAVTLAYQHNNSGFVGYLAPTMRQGQPYPANYPYPLIGKSAVTSVTQKKFLCDRVMWRIPFSSNFMSMGALTDLGQNMLYANSAHALDMNFEVDPMDESTLLYVVFEVFDVVRVHQPHRGVIEAVYLRTPFSAGNATT

SEQ ID NO: 21 - protein, 942 aa, synthetic construct
MATPSMLPQWAYMHIAGQDASEYLSPGLVQFARATDTYFSLGNKFRNPTVAPTHDVTTDRSQRLTLRFVPVDREDNTYSYKVRYTLAVGDNRVLDMASTYFDIRGVLDRGPSFKPYSGTAYNSLAPKGAPNSSQWEQKKAGNGDTMETHTFGVAPMGGENITIDGLQIGTKATAKQKKPIYADKTFQPEPQVGEENWQETESFYGGRALKKDTSMKPCYGSYARPTNVKGGQAKLKVGADGVPTKEFDIDLAFFDTPGGTVNGQDEYKADIVMYTENTYLETPDTHVVYKPGKDDASSEINLVQQSMPNRPNYIGFRDNFIGLMYYNSTGNMGVLAGQASQLNAVVDLQDRNTELSYQLLLDSLGDRTRYFSMWNQAVDSYDPDVRIIENHGVEDELPNYCFPLDGSGTNAAYQGVKVKNGNKGNVQSQWENDDTVAARNQLCKGNIFAMEINLQANLWRSFLYSNVALYLPDSYKYTPANITLPTNTNTYDYMNGRVVPPSLVDAYINIGARWSLDPMDNVNPFNHHRNAGLRYRSMLLGNGRYVPFHIQVPQKFFAIKSLLLLPGSYTYEWNFRKDVNMILQSSLGNDLRTDGASISFTSINLYATFFPMAHNTASTLEAMLRNDTNDQSFNDYLSAANMLYPIPANATNVPISIPSRNWAAFRGWSFTRLKTKETPSLGSGFDPYFVYSGSIPYLDGTFYLNHTFKKVSITFDSSVSWPGNDRLLTPNEFEIKRTVDGEGYNVAQCNMTKDWFLVQMLAHYNIGYQGFYVPEGYKDRMYSFFRNFQPMSRQVVDEVNYKDYQAVTLAYQHNNSGFVGYLAPTMRQGQPYPANYPYPLIGKSAVTSVTQKKFLCDRVMWRIPFSSNFMSMGALTDLGQNMLYANSAHALDMNFEVDPMDESTLLYVVFEVFDVVRVHQPHRGVIEAVYLRTPFSAGNATT

SEQ ID NO: 22 - protein, 942 aa, synthetic construct
MATPSMLPQWAYMHIAGQDASEYLSPGLVQFARATDTYFSLGNKFRNPTVAPTHDVTTDRSQRLTLRFVPVDREDNTYSYKVRYTLAVGDNRVLDMASTYFDIRGVLDRGPSFKPYSGTAYNSLAPKGAPNSSQWEQKKAGNGDTMETHTFGVAPMGGENITIDGLQIGTKATAKQNKPIYADKTFQPEPQVGEENWQETESFYGGRALKKDTSMKPCYGSYARPTNVKGGQAKLKVGADGVPTKEFDIDLAFFDTPGGTVNGQDEYKADIVMYTENTYLETPDTHVVYKPGKDDASSEINLVQQSMPNRPNYIGFRDNFIGLMYYNSTGNMGVLAGQASQLNAVVDLQDRNTELSYQLLLDSLGDRTRYFSMWNQAVDSYDPDVRIIENHGVEDELPNYCFPLDGSGTNAAYQGVKVKNGNNGNVKSKWENDDTVAARNQLCKGNIFAMEINLQANLWRSFLYSNVALYLPDSYKYTPANITLPTNTNTYDYMNGRVVPPSLVDAYINIGARWSLDPMDNVNPFNHHRNAGLRYRSMLLGNGRYVPFHIQVPQKFFAIKSLLLLPGSYTYEWNFRKDVNMILQSSLGNDLRTDGASISFTSINLYATFFPMAHNTASTLEAMLRNDTNDQSFNDYLSAANMLYPIPANATNVPISIPSRNWAAFRGWSFTRLKTKETPSLGSGFDPYFVYSGSIPYLDGTFYLNHTFKKVSITFDSSVSWPGNDRLLTPNEFEIKRTVDGEGYNVAQCNMTKDWFLVQMLAHYNIGYQGFYVPEGYKDRMYSFFRNFQPMSRQVVDEVNYKDYQAVTLAYQHNNSGFVGYLAPTMRQGQPYPANYPYPLIGKSAVTSVTQKKFLCDRVMWRIPFSSNFMSMGALTDLGQNMLYANSAHALDMNFEVDPMDESTLLYVVFEVFDVVRVHQPHRGVIEAVYLRTPFSAGNATT

SEQ ID NO: 23 - protein, 942 aa, synthetic construct
MATPSMLPQWAYMHIAGQDASEYLSPGLVQFARATDTYFSLGNKFRNPTVAPTHDVTTDRSQRLTLRFVPVDREDNTYSYKVRYTLAVGDNRVLDMASTYFDIRGVLDRGPSFKPYSGTAYNSLAPKGAPNSSQWEQKKAGNGDTMETHTFGVAPMGGENITIDGLQIGTKATAKQNKPIYADKTFQPEPQVGEENWQETESFYGGRALKKDTSMKPCYGSYARPTNVKGGQAKLKVGADGVPTKEFDIDLAFFDTPGGTVNGQDEYKADIVMYTENTYLETPDTHVVYKPGKDDASSEINLVQQSMPNRPNYIGFRDNFIGLMYYNSTGNMGVLAGQASQLNAVVDLQDRNTELSYQLLLDSLGDRTRYFSMWNQAVDSYDPDVRIIENHGVEDELPNYCFPLDGSGTNAAYQGVKVKNGNKGKVQSQWENDDTVAARNQLCKGNIFAMEINLQANLWRSFLYSNVALYLPDSYKYTPANITLPTNTNTYDYMNGRVVPPSLVDAYINIGARWSLDPMDNVNPFNHHRNAGLRYRSMLLGNGRYVPFHIQVPQKFFAIKSLLLLPGSYTYEWNFRKDVNMILQSSLGNDLRTDGASISFTSINLYATFFPMAHNTASTLEAMLRNDTNDQSFNDYLSAANMLYPIPANATNVPISIPSRNWAAFRGWSFTRLKTKETPSLGSGFDPYFVYSGSIPYLDGTFYLNHTFKKVSITFDSSVSWPGNDRLLTPNEFEIKRTVDGEGYNVAQCNMTKDWFLVQMLAHYNIGYQGFYVPEGYKDRMYSFFRNFQPMSRQVVDEVNYKDYQAVTLAYQHNNSGFVGYLAPTMRQGQPYPANYPYPLIGKSAVTSVTQKKFLCDRVMWRIPFSSNFMSMGALTDLGQNMLYANSAHALDMNFEVDPMDESTLLYVVFEVFDVVRVHQPHRGVIEAVYLRTPFSAGNATT

SEQ ID NO: 24 - protein, 942 aa, synthetic construct
MATPSMLPQWAYMHIAGQDASEYLSPGLVQFARATDTYFSLGNKFRNPTVAPTHDVTTDRSQRLTLRFVPVDREDNTYSYKVRYTLAVGDNRVLDMASTYFDIRGVLDRGPSFKPYSGTAYNSLAPKGAPNSSQWEQKKAGNGDTMETHTFGVAPMGGENITIDGLQIGTKATAKQKKPIYADKTFQPEPQVGEENWQETESFYGGRALKKDTSMKPCYGSYARPTNVKGGQAKLKVGADGVPTKEFDIDLAFFDTPGGTVNGQDEYKADIVMYTENTYLETPDTHVVYKPGKDDASSEINLVQQSMPNRPNYIGFRDNFIGLMYYNSTGNMGVLAGQASQLNAVVDLQDRNTELSYQLLLDSLGDRTRYFSMWNQAVDSYDPDVRIIENHGVEDELPNYCFPLDGSGTNAAYQGVKVKNGNKGKVQSQWENDDTVAARNQLCKGNIFAMEINLQANLWRSFLYSNVALYLPDSYKYTPANITLPTNTNTYDYMNGRVVPPSLVDAYINIGARWSLDPMDNVNPFNHHRNAGLRYRSMLLGNGRYVPFHIQVPQKFFAIKSLLLLPGSYTYEWNFRKDVNMILQSSLGNDLRTDGASISFTSINLYATFFPMAHNTASTLEAMLRNDTNDQSFNDYLSAANMLYPIPANATNVPISIPSRNWAAFRGWSFTRLKTKETPSLGSGFDPYFVYSGSIPYLDGTFYLNHTFKKVSITFDSSVSWPGNDRLLTPNEFEIKRTVDGEGYNVAQCNMTKDWFLVQMLAHYNIGYQGFYVPEGYKDRMYSFFRNFQPMSRQVVDEVNYKDYQAVTLAYQHNNSGFVGYLAPTMRQGQPYPANYPYPLIGKSAVTSVTQKKFLCDRVMWRIPFSSNFMSMGALTDLGQNMLYANSAHALDMNFEVDPMDESTLLYVVFEVFDVVRVHQPHRGVIEAVYLRTPFSAGNATT

SEQ ID NO: 25 - protein, 942 aa, synthetic construct
MATPSMLPQWAYMHIAGQDASEYLSPGLVQFARATDTYFSLGNKFRNPTVAPTHDVTTDRSQRLTLRFVPVDREDNTYSYKVRYTLAVGDNRVLDMASTYFDIRGVLDRGPSFKPYSGTAYNSLAPKGAPNSSQWEQKKAGNGDTMETHTFGVAPMGGENITIDGLQIGTKATAKQKKPIYADKTFQPEPQVGEENWQETESFYGGRALKKDTSMKPCYGSYARPTNVKGGQAKLKVGADGVPTKEFDIDLAFFDTPGGTVNGQDEYKADIVMYTENTYLETPDTHVVYKPGKDDASSEINLVQQSMPNRPNYIGFRDNFIGLMYYNSTGNMGVLAGQASQLNAVVDLQDRNTELSYQLLLDSLGDRTRYFSMWNQAVDSYDPDVRIIENHGVEDELPNYCFPLDGSGTNAAYQGVKVKNGNNGNVKSKWENDDTVAARNQLCKGNIFAMEINLQANLWRSFLYSNVALYLPDSYKYTPANITLPTNTNTYDYMNGRVVPPSLVDAYINIGARWSLDPMDNVNPFNHHRNAGLRYRSMLLGNGRYVPFHIQVPQKFFAIKSLLLLPGSYTYEWNFRKDVNMILQSSLGNDLRTDGASISFTSINLYATFFPMAHNTASTLEAMLRNDTNDQSFNDYLSAANMLYPIPANATNVPISIPSRNWAAFRGWSFTRLKTKETPSLGSGFDPYFVYSGSIPYLDGTFYLNHTFKKVSITFDSSVSWPGNDRLLTPNEFEIKRTVDGEGYNVAQCNMTKDWFLVQMLAHYNIGYQGFYVPEGYKDRMYSFFRNFQPMSRQVVDEVNYKDYQAVTLAYQHNNSGFVGYLAPTMRQGQPYPANYPYPLIGKSAVTSVTQKKFLCDRVMWRIPFSSNFMSMGALTDLGQNMLYANSAHALDMNFEVDPMDESTLLYVVFEVFDVVRVHQPHRGVIEAVYLRTPFSAGNATT

SEQ ID NO: 26 - protein, 942 aa, synthetic construct
MATPSMLPQWAYMHIAGQDASEYLSPGLVQFARATDTYFSLGNKFRNPTVAPTHDVTTDRSQRLTLRFVPVDREDNTYSYKVRYTLAVGDNRVLDMASTYFDIRGVLDRGPSFKPYSGTAYNSLAPKGAPNSSQWEQKKAGNGDTMETHTFGVAPMGGENITIDGLQIGTKATANQKKPIYADKTFQPEPQVGEENWQETESFYGGRALKKDTSMKPCYGSYARPTNVKGGQAKLKVGADGVPTKEFDIDLAFFDTPGGTVNGQDEYKADIVMYTENTYLETPDTHVVYKPGKDDASSEINLVQQSMPNRPNYIGFRDNFIGLMYYNSTGNMGVLAGQASQLNAVVDLQDRNTELSYQLLLDSLGDRTRYFSMWNQAVDSYDPDVRIIENHGVEDELPNYCFPLDGSGTNAAYQGVKVKNGNKGKVKSQWENDDTVAARNQLCKGNIFAMEINLQANLWRSFLYSNVALYLPDSYKYTPANITLPTNTNTYDYMNGRVVPPSLVDAYINIGARWSLDPMDNVNPFNHHRNAGLRYRSMLLGNGRYVPFHIQVPQKFFAIKSLLLLPGSYTYEWNFRKDVNMILQSSLGNDLRTDGASISFTSINLYATFFPMAHNTASTLEAMLRNDTNDQSFNDYLSAANMLYPIPANATNVPISIPSRNWAAFRGWSFTRLKTKETPSLGSGFDPYFVYSGSIPYLDGTFYLNHTFKKVSITFDSSVSWPGNDRLLTPNEFEIKRTVDGEGYNVAQCNMTKDWFLVQMLAHYNIGYQGFYVPEGYKDRMYSFFRNFQPMSRQVVDEVNYKDYQAVTLAYQHNNSGFVGYLAPTMRQGQPYPANYPYPLIGKSAVTSVTQKKFLCDRVMWRIPFSSNFMSMGALTDLGQNMLYANSAHALDMNFEVDPMDESTLLYVVFEVFDVVRVHQPHRGVIEAVYLRTPFSAGNATT

SEQ ID NO: 27 - protein, 942 aa, synthetic construct
MATPSMLPQWAYMHIAGQDASEYLSPGLVQFARATDTYFSLGNKFRNPTVAPTHDVTTDRSQRLTLRFVPVDREDNTYSYKVRYTLAVGDNRVLDMASTYFDIRGVLDRGPSFKPYSGTAYNSLAPKGAPNSSQWEQKKAGNGDTMETHTFGVAPMGGENITIDGLQIGTKATAKQKKPIYADKTFQPEPQVGEENWQETESFYGGRALKKDTSMKPCYGSYARPTNVKGGQAKLKVGADGVPTKEFDIDLAFFDTPGGTVNGQDEYKADIVMYTENTYLETPDTHVVYKPGKDDASSEINLVQQSMPNRPNYIGFRDNFIGLMYYNSTGNMGVLAGQASQLNAVVDLQDRNTELSYQLLLDSLGDRTRYFSMWNQAVDSYDPDVRIIENHGVEDELPNYCFPLDGSGTNAAYQGVKVKNGNKGKVKSQWENDDTVAARNQLCKGNIFAMEINLQANLWRSFLYSNVALYLPDSYKYTPANITLPTNTNTYDYMNGRVVPPSLVDAYINIGARWSLDPMDNVNPFNHHRNAGLRYRSMLLGNGRYVPFHIQVPQKFFAIKSLLLLPGSYTYEWNFRKDVNMILQSSLGNDLRTDGASISFTSINLYATFFPMAHNTASTLEAMLRNDTNDQSFNDYLSAANMLYPIPANATNVPISIPSRNWAAFRGWSFTRLKTKETPSLGSGFDPYFVYSGSIPYLDGTFYLNHTFKKVSITFDSSVSWPGNDRLLTPNEFEIKRTVDGEGYNVAQCNMTKDWFLVQMLAHYNIGYQGFYVPEGYKDRMYSFFRNFQPMSRQVVDEVNYKDYQAVTLAYQHNNSGFVGYLAPTMRQGQPYPANYPYPLIGKSAVTSVTQKKFLCDRVMWRIPFSSNFMSMGALTDLGQNMLYANSAHALDMNFEVDPMDESTLLYVVFEVFDVVRVHQPHRGVIEAVYLRTPFSAGNATT

SEQ ID NO: 28 - protein, 942 aa, synthetic construct
MATPSMLPQWAYMHIAGQDASEYLSPGLVQFARATDTYFSLGNKFRNPTVAPTHDVTTDRSQRLTLRFVPVDREDNTYSYKVRYTLAVGDNRVLDMASTYFDIRGVLDRGPSFKPYSGTAYNSLAPKGAPNSSQWEQKKAGNGDTMETHTFGVAPMGGENITIDGLQIGTKATAKQKKPIYADKTFQPEPQVGEENWQETESFYGGRALKKDTSMKPCYGSYARPTNVKGGQAKLKVGADGVPTKEFDIDLAFFDTPGGTVNGQDEYKADIVMYTENTYLETPDTHVVYKPGKDDASSEINLVQQSMPNRPNYIGFRDNFIGLMYYNSTGNMGVLAGQASQLNAVVDLQDRNTELSYQLLLDSLGDRTRYFSMWNQAVDSYDPDVRIIENHGVEDELPNYCFPLDGSGTNAAYQGVKVKNGNKGKVQSKWENDDTVAARNQLCKGNIFAMEINLQANLWRSFLYSNVALYLPDSYKYTPANITLPTNTNTYDYMNGRVVPPSLVDAYINIGARWSLDPMDNVNPFNHHRNAGLRYRSMLLGNGRYVPFHIQVPQKFFAIKSLLLLPGSYTYEWNFRKDVNMILQSSLGNDLRTDGASISFTSINLYATFFPMAHNTASTLEAMLRNDTNDQSFNDYLSAANMLYPIPANATNVPISIPSRNWAAFRGWSFTRLKTKETPSLGSGFDPYFVYSGSIPYLDGTFYLNHTFKKVSITFDSSVSWPGNDRLLTPNEFEIKRTVDGEGYNVAQCNMTKDWFLVQMLAHYNIGYQGFYVPEGYKDRMYSFFRNFQPMSRQVVDEVNYKDYQAVTLAYQHNNSGFVGYLAPTMRQGQPYPANYPYPLIGKSAVTSVTQKKFLCDRVMWRIPFSSNFMSMGALTDLGQNMLYANSAHALDMNFEVDPMDESTLLYVVFEVFDVVRVHQPHRGVIEAVYLRTPFSAGNATT

SEQ ID NO: 29 - protein, 942 aa, synthetic construct
MATPSMLPQWAYMHIAGQDASEYLSPGLVQFARATDTYFSLGNKFRNPTVAPTHDVTTDRSQRLTLRFVPVDREDNTYSYKVRYTLAVGDNRVLDMASTYFDIRGVLDRGPSFKPYSGTAYNSLAPKGAPNSSQWEQKKAGNGDTMETHTFGVAPMGGENITIDGLQIGTKATAKQKKPIYADKTFQPEPQVGEENWQETESFYGGRALKKDTSMKPCYGSYARPTNVKGGQAKLKVGADGVPTKEFDIDLAFFDTPGGTVNGQDEYKADIVMYTENTYLETPDTHVVYKPGKDDASSEINLVQQSMPNRPNYIGFRDNFIGLMYYNSTGNMGVLAGQASQLNAVVDLQDRNTELSYQLLLDSLGDRTRYFSMWNQAVDSYDPDVRIIENHGVEDELPNYCFPLDGSGTNAAYQGVKVKNGNKGNVKSKWENDDTVAARNQLCKGNIFAMEINLQANLWRSFLYSNVALYLPDSYKYTPANITLPTNTNTYDYMNGRVVPPSLVDAYINIGARWSLDPMDNVNPFNHHRNAGLRYRSMLLGNGRYVPFHIQVPQKFFAIKSLLLLPGSYTYEWNFRKDVNMILQSSLGNDLRTDGASISFTSINLYATFFPMAHNTASTLEAMLRNDTNDQSFNDYLSAANMLYPIPANATNVPISIPSRNWAAFRGWSFTRLKTKETPSLGSGFDPYFVYSGSIPYLDGTFYLNHTFKKVSITFDSSVSWPGNDRLLTPNEFEIKRTVDGEGYNVAQCNMTKDWFLVQMLAHYNIGYQGFYVPEGYKDRMYSFFRNFQPMSRQVVDEVNYKDYQAVTLAYQHNNSGFVGYLAPTMRQGQPYPANYPYPLIGKSAVTSVTQKKFLCDRVMWRIPFSSNFMSMGALTDLGQNMLYANSAHALDMNFEVDPMDESTLLYVVFEVFDVVRVHQPHRGVIEAVYLRTPFSAGNATT

SEQ ID NO: 30 - protein, 942 aa, synthetic construct
MATPSMLPQWAYMHIAGQDASEYLSPGLVQFARATDTYFSLGNKFRNPTVAPTHDVTTDRSQRLTLRFVPVDREDNTYSYKVRYTLAVGDNRVLDMASTYFDIRGVLDRGPSFKPYSGTAYNSLAPKGAPNSSQWEQKKAGNGDTMETHTFGVAPMGGENITIDGLQIGTKATAKQKKPIYADKTFQPEPQVGEENWQETESFYGGRALKKDTSMKPCYGSYARPTNVKGGQAKLKVGADGVPTKEFDIDLAFFDTPGGTVNGQDEYKADIVMYTENTYLETPDTHVVYKPGKDDASSEINLVQQSMPNRPNYIGFRDNFIGLMYYNSTGNMGVLAGQASQLNAVVDLQDRNTELSYQLLLDSLGDRTRYFSMWNQAVDSYDPDVRIIENHGVEDELPNYCFPLDGSGTNAAYQGVKVKNGNNGKVKSKWENDDTVAARNQLCKGNIFAMEINLQANLWRSFLYSNVALYLPDSYKYTPANITLPTNTNTYDYMNGRVVPPSLVDAYINIGARWSLDPMDNVNPFNHHRNAGLRYRSMLLGNGRYVPFHIQVPQKFFAIKSLLLLPGSYTYEWNFRKDVNMILQSSLGNDLRTDGASISFTSINLYATFFPMAHNTASTLEAMLRNDTNDQSFNDYLSAANMLYPIPANATNVPISIPSRNWAAFRGWSFTRLKTKETPSLGSGFDPYFVYSGSIPYLDGTFYLNHTFKKVSITFDSSVSWPGNDRLLTPNEFEIKRTVDGEGYNVAQCNMTKDWFLVQMLAHYNIGYQGFYVPEGYKDRMYSFFRNFQPMSRQVVDEVNYKDYQAVTLAYQHNNSGFVGYLAPTMRQGQPYPANYPYPLIGKSAVTSVTQKKFLCDRVMWRIPFSSNFMSMGALTDLGQNMLYANSAHALDMNFEVDPMDESTLLYVVFEVFDVVRVHQPHRGVIEAVYLRTPFSAGNATT

SEQ ID NO: 31 - protein, 942 aa, synthetic construct
MATPSMLPQWAYMHIAGQDASEYLSPGLVQFARATDTYFSLGNKFRNPTVAPTHDVTTDRSQRLTLRFVPVDREDNTYSYKVRYTLAVGDNRVLDMASTYFDIRGVLDRGPSFKPYSGTAYNSLAPKGAPNSSQWEQKKAGNGDTMETHTFGVAPMGGENITIDGLQIGTVATAVQVKPIYADKTFQPEPQVGEENWQETESFYGGRALKKDTSMKPCYGSYARPTNVKGGQAKLKVGADGVPTKEFDIDLAFFDTPGGTVNGQDEYKADIVMYTENTYLETPDTHVVYKPGKDDASSEINLVQQSMPNRPNYIGFRDNFIGLMYYNSTGNMGVLAGQASQLNAVVDLQDRNTELSYQLLLDSLGDRTRYFSMWNQAVDSYDPDVRIIENHGVEDELPNYCFPLDGSGTNAAYQGVKVKNGNVGVVQSQWENDDTVAARNQLCKGNIFAMEINLQANLWRSFLYSNVALYLPDSYKYTPANITLPTNTNTYDYMNGRVVPPSLVDAYINIGARWSLDPMDNVNPFNHHRNAGLRYRSMLLGNGRYVPFHIQVPQKFFAIKSLLLLPGSYTYEWNFRKDVNMILQSSLGNDLRTDGASISFTSINLYATFFPMAHNTASTLEAMLRNDTNDQSFNDYLSAANMLYPIPANATNVPISIPSRNWAAFRGWSFTRLKTKETPSLGSGFDPYFVYSGSIPYLDGTFYLNHTFKKVSITFDSSVSWPGNDRLLTPNEFEIKRTVDGEGYNVAQCNMTKDWFLVQMLAHYNIGYQGFYVPEGYKDRMYSFFRNFQPMSRQVVDEVNYKDYQAVTLAYQHNNSGFVGYLAPTMRQGQPYPANYPYPLIGKSAVTSVTQKKFLCDRVMWRIPFSSNFMSMGALTDLGQNMLYANSAHALDMNFEVDPMDESTLLYVVFEVFDVVRVHQPHRGVIEAVYLRTPFSAGNATT

SEQ ID NO: 32 - protein, 942 aa, synthetic construct
MATPSMLPQWAYMHIAGQDASEYLSPGLVQFARATDTYFSLGNKFRNPTVAPTHDVTTDRSQRLTLRFVPVDREDNTYSYKVRYTLAVGDNRVLDMASTYFDIRGVLDRGPSFKPYSGTAYNSLAPKGAPNSSQWEQKKAGNGDTMETHTFGVAPMGGENITIDGLQIGTTATATQTKPIYADKTFQPEPQVGEENWQETESFYGGRALKKDTSMKPCYGSYARPTNVKGGQAKLKVGADGVPTKEFDIDLAFFDTPGGTVNGQDEYKADIVMYTENTYLETPDTHVVYKPGKDDASSEINLVQQSMPNRPNYIGFRDNFIGLMYYNSTGNMGVLAGQASQLNAVVDLQDRNTELSYQLLLDSLGDRTRYFSMWNQAVDSYDPDVRIIENHGVEDELPNYCFPLDGSGTNAAYQGVKVKNGNTGTVQSQWENDDTVAARNQLCKGNIFAMEINLQANLWRSFLYSNVALYLPDSYKYTPANITLPTNTNTYDYMNGRVVPPSLVDAYINIGARWSLDPMDNVNPFNHHRNAGLRYRSMLLGNGRYVPFHIQVPQKFFAIKSLLLLPGSYTYEWNFRKDVNMILQSSLGNDLRTDGASISFTSINLYATFFPMAHNTASTLEAMLRNDTNDQSFNDYLSAANMLYPIPANATNVPISIPSRNWAAFRGWSFTRLKTKETPSLGSGFDPYFVYSGSIPYLDGTFYLNHTFKKVSITFDSSVSWPGNDRLLTPNEFEIKRTVDGEGYNVAQCNMTKDWFLVQMLAHYNIGYQGFYVPEGYKDRMYSFFRNFQPMSRQVVDEVNYKDYQAVTLAYQHNNSGFVGYLAPTMRQGQPYPANYPYPLIGKSAVTSVTQKKFLCDRVMWRIPFSSNFMSMGALTDLGQNMLYANSAHALDMNFEVDPMDESTLLYVVFEVFDVVRVHQPHRGVIEAVYLRTPFSAGNATT

SEQ ID NO: 33 - protein, 942 aa, synthetic construct
MATPSMLPQWAYMHIAGQDASEYLSPGLVQFARATDTYFSLGNKFRNPTVAPTHDVTTDRSQRLTLRFVPVDREDNTYSYKVRYTLAVGDNRVLDMASTYFDIRGVLDRGPSFKPYSGTAYNSLAPKGAPNSSQWEQKKAGNGDTMETHTFGVAPMGGENITIDGLQIGTNATANQNKPIYADKTFQPEPQVGEENWQETESFYGGRALKKDTSMKPCYGSYARPTNVKGGQAKLKVGADGVPTKEFDIDLAFFDTPGGTVNGQDEYKADIVMYTENTYLETPDTHVVYKPGKDDASSEINLVQQSMPNRPNYIGFRDNFIGLMYYNSTGNMGVLAGQASQLNAVVDLQDRNTELSYQLLLDSLGDRTRYFSMWNQAVDSYDPDVRIIENHGVEDELPNYCFPLDGSGTNAAYQGVKVKNGNNGNVLSLWENDDTVAARNQLCKGNIFAMEINLQANLWRSFLYSNVALYLPDSYKYTPANITLPTNTNTYDYMNGRVVPPSLVDAYINIGARWSLDPMDNVNPFNHHRNAGLRYRSMLLGNGRYVPFHIQVPQKFFAIKSLLLLPGSYTYEWNFRKDVNMILQSSLGNDLRTDGASISFTSINLYATFFPMAHNTASTLEAMLRNDTNDQSFNDYLSAANMLYPIPANATNVPISIPSRNWAAFRGWSFTRLKTKETPSLGSGFDPYFVYSGSIPYLDGTFYLNHTFKKVSITFDSSVSWPGNDRLLTPNEFEIKRTVDGEGYNVAQCNMTKDWFLVQMLAHYNIGYQGFYVPEGYKDRMYSFFRNFQPMSRQVVDEVNYKDYQAVTLAYQHNNSGFVGYLAPTMRQGQPYPANYPYPLIGKSAVTSVTQKKFLCDRVMWRIPFSSNFMSMGALTDLGQNMLYANSAHALDMNFEVDPMDESTLLYVVFEVFDVVRVHQPHRGVIEAVYLRTPFSAGNATT

SEQ ID NO: 34 - protein, 942 aa, synthetic construct
MATPSMLPQWAYMHIAGQDASEYLSPGLVQFARATDTYFSLGNKFRNPTVAPTHDVTTDRSQRLTLRFVPVDREDNTYSYKVRYTLAVGDNRVLDMASTYFDIRGVLDRGPSFKPYSGTAYNSLAPKGAPNSSQWEQKKAGNGDTMETHTFGVAPMGGENITIDGLQIGTVATAVQVKPIYADKTFQPEPQVGEENWQETESFYGGRALKKDTSMKPCYGSYARPTNVKGGQAKLKVGADGVPTKEFDIDLAFFDTPGGTVNGQDEYKADIVMYTENTYLETPDTHVVYKPGKDDASSEINLVQQSMPNRPNYIGFRDNFIGLMYYNSTGNMGVLAGQASQLNAVVDLQDRNTELSYQLLLDSLGDRTRYFSMWNQAVDSYDPDVRIIENHGVEDELPNYCFPLDGSGTNAAYQGVKVKNGNVGVVLSLWENDDTVAARNQLCKGNIFAMEINLQANLWRSFLYSNVALYLPDSYKYTPANITLPTNTNTYDYMNGRVVPPSLVDAYINIGARWSLDPMDNVNPFNHHRNAGLRYRSMLLGNGRYVPFHIQVPQKFFAIKSLLLLPGSYTYEWNFRKDVNMILQSSLGNDLRTDGASISFTSINLYATFFPMAHNTASTLEAMLRNDTNDQSFNDYLSAANMLYPIPANATNVPISIPSRNWAAFRGWSFTRLKTKETPSLGSGFDPYFVYSGSIPYLDGTFYLNHTFKKVSITFDSSVSWPGNDRLLTPNEFEIKRTVDGEGYNVAQCNMTKDWFLVQMLAHYNIGYQGFYVPEGYKDRMYSFFRNFQPMSRQVVDEVNYKDYQAVTLAYQHNNSGFVGYLAPTMRQGQPYPANYPYPLIGKSAVTSVTQKKFLCDRVMWRIPFSSNFMSMGALTDLGQNMLYANSAHALDMNFEVDPMDESTLLYVVFEVFDVVRVHQPHRGVIEAVYLRTPFSAGNATT

SEQ ID NO: 35 - protein, 942 aa, synthetic construct
MATPSMLPQWAYMHIAGQDASEYLSPGLVQFARATDTYFSLGNKFRNPTVAPTHDVTTDRSQRLTLRFVPVDREDNTYSYKVRYTLAVGDNRVLDMASTYFDIRGVLDRGPSFKPYSGTAYNSLAPKGAPNSSQWEQKKAGNGDTMETHTFGVAPMGGENITIDGLQIGTTATATQTKPIYADKTFQPEPQVGEENWQETESFYGGRALKKDTSMKPCYGSYARPTNVKGGQAKLKVGADGVPTKEFDIDLAFFDTPGGTVNGQDEYKADIVMYTENTYLETPDTHVVYKPGKDDASSEINLVQQSMPNRPNYIGFRDNFIGLMYYNSTGNMGVLAGQASQLNAVVDLQDRNTELSYQLLLDSLGDRTRYFSMWNQAVDSYDPDVRIIENHGVEDELPNYCFPLDGSGTNAAYQGVKVKNGNTGTVLSLWENDDTVAARNQLCKGNIFAMEINLQANLWRSFLYSNVALYLPDSYKYTPANITLPTNTNTYDYMNGRVVPPSLVDAYINIGARWSLDPMDNVNPFNHHRNAGLRYRSMLLGNGRYVPFHIQVPQKFFAIKSLLLLPGSYTYEWNFRKDVNMILQSSLGNDLRTDGASISFTSINLYATFFPMAHNTASTLEAMLRNDTNDQSFNDYLSAANMLYPIPANATNVPISIPSRNWAAFRGWSFTRLKTKETPSLGSGFDPYFVYSGSIPYLDGTFYLNHTFKKVSITFDSSVSWPGNDRLLTPNEFEIKRTVDGEGYNVAQCNMTKDWFLVQMLAHYNIGYQGFYVPEGYKDRMYSFFRNFQPMSRQVVDEVNYKDYQAVTLAYQHNNSGFVGYLAPTMRQGQPYPANYPYPLIGKSAVTSVTQKKFLCDRVMWRIPFSSNFMSMGALTDLGQNMLYANSAHALDMNFEVDPMDESTLLYVVFEVFDVVRVHQPHRGVIEAVYLRTPFSAGNATT

SEQ ID NO: 36 - protein, 942 aa, synthetic construct
MATPSMLPQWAYMHIAGQDASEYLSPGLVQFARATDTYFSLGNKFRNPTVAPTHDVTTDRSQRLTLRFVPVDREDNTYSYKVRYTLAVGDNRVLDMASTYFDIRGVLDRGPSFKPYSGTAYNSLAPKGAPNSSQWEQKKAGNGDTMETHTFGVAPMGGENITIDGLQIGTNATANQNKPIYADKTFQPEPQVGEENWQETESFYGGRALKKDTSMKPCYGSYARPTNVKGGQAKLKVGADGVPTKEFDIDLAFFDTPGGTVNGQDEYKADIVMYTENTYLETPDTHVVYKPGKDDASSEINLVQQSMPNRPNYIGFRDNFIGLMYYNSTGNMGVLAGQASQLNAVVDLQDRNTELSYQLLLDSLGDRTRYFSMWNQAVDSYDPDVRIIENHGVEDELPNYCFPLDGSGTNAAYQGVKVKNGNNGNVISIWENDDTVAARNQLCKGNIFAMEINLQANLWRSFLYSNVALYLPDSYKYTPANITLPTNTNTYDYMNGRVVPPSLVDAYINIGARWSLDPMDNVNPFNHHRNAGLRYRSMLLGNGRYVPFHIQVPQKFFAIKSLLLLPGSYTYEWNFRKDVNMILQSSLGNDLRTDGASISFTSINLYATFFPMAHNTASTLEAMLRNDTNDQSFNDYLSAANMLYPIPANATNVPISIPSRNWAAFRGWSFTRLKTKETPSLGSGFDPYFVYSGSIPYLDGTFYLNHTFKKVSITFDSSVSWPGNDRLLTPNEFEIKRTVDGEGYNVAQCNMTKDWFLVQMLAHYNIGYQGFYVPEGYKDRMYSFFRNFQPMSRQVVDEVNYKDYQAVTLAYQHNNSGFVGYLAPTMRQGQPYPANYPYPLIGKSAVTSVTQKKFLCDRVMWRIPFSSNFMSMGALTDLGQNMLYANSAHALDMNFEVDPMDESTLLYVVFEVFDVVRVHQPHRGVIEAVYLRTPFSAGNATT

SEQ ID NO: 37 - protein, 942 aa, synthetic construct
MATPSMLPQWAYMHIAGQDASEYLSPGLVQFARATDTYFSLGNKFRNPTVAPTHDVTTDRSQRLTLRFVPVDREDNTYSYKVRYTLAVGDNRVLDMASTYFDIRGVLDRGPSFKPYSGTAYNSLAPKGAPNSSQWEQKKAGNGDTMETHTFGVAPMGGENITIDGLQIGTVATAVQVKPIYADKTFQPEPQVGEENWQETESFYGGRALKKDTSMKPCYGSYARPTNVKGGQAKLKVGADGVPTKEFDIDLAFFDTPGGTVNGQDEYKADIVMYTENTYLETPDTHVVYKPGKDDASSEINLVQQSMPNRPNYIGFRDNFIGLMYYNSTGNMGVLAGQASQLNAVVDLQDRNTELSYQLLLDSLGDRTRYFSMWNQAVDSYDPDVRIIENHGVEDELPNYCFPLDGSGTNAAYQGVKVKNGNVGVVISIWENDDTVAARNQLCKGNIFAMEINLQANLWRSFLYSNVALYLPDSYKYTPANITLPTNTNTYDYMNGRVVPPSLVDAYINIGARWSLDPMDNVNPFNHHRNAGLRYRSMLLGNGRYVPFHIQVPQKFFAIKSLLLLPGSYTYEWNFRKDVNMILQSSLGNDLRTDGASISFTSINLYATFFPMAHNTASTLEAMLRNDTNDQSFNDYLSAANMLYPIPANATNVPISIPSRNWAAFRGWSFTRLKTKETPSLGSGFDPYFVYSGSIPYLDGTFYLNHTFKKVSITFDSSVSWPGNDRLLTPNEFEIKRTVDGEGYNVAQCNMTKDWFLVQMLAHYNIGYQGFYVPEGYKDRMYSFFRNFQPMSRQVVDEVNYKDYQAVTLAYQHNNSGFVGYLAPTMRQGQPYPANYPYPLIGKSAVTSVTQKKFLCDRVMWRIPFSSNFMSMGALTDLGQNMLYANSAHALDMNFEVDPMDESTLLYVVFEVFDVVRVHQPHRGVIEAVYLRTPFSAGNATT

SEQ ID NO: 38 - protein, 942 aa, synthetic construct
MATPSMLPQWAYMHIAGQDASEYLSPGLVQFARATDTYFSLGNKFRNPTVAPTHDVTTDRSQRLTLRFVPVDREDNTYSYKVRYTLAVGDNRVLDMASTYFDIRGVLDRGPSFKPYSGTAYNSLAPKGAPNSSQWEQKKAGNGDTMETHTFGVAPMGGENITIDGLQIGTTATATQTKPIYADKTFQPEPQVGEENWQETESFYGGRALKKDTSMKPCYGSYARPTNVKGGQAKLKVGADGVPTKEFDIDLAFFDTPGGTVNGQDEYKADIVMYTENTYLETPDTHVVYKPGKDDASSEINLVQQSMPNRPNYIGFRDNFIGLMYYNSTGNMGVLAGQASQLNAVVDLQDRNTELSYQLLLDSLGDRTRYFSMWNQAVDSYDPDVRIIENHGVEDELPNYCFPLDGSGTNAAYQGVKVKNGNTGTVISIWENDDTVAARNQLCKGNIFAMEINLQANLWRSFLYSNVALYLPDSYKYTPANITLPTNTNTYDYMNGRVVPPSLVDAYINIGARWSLDPMDNVNPFNHHRNAGLRYRSMLLGNGRYVPFHIQVPQKFFAIKSLLLLPGSYTYEWNFRKDVNMILQSSLGNDLRTDGASISFTSINLYATFFPMAHNTASTLEAMLRNDTNDQSFNDYLSAANMLYPIPANATNVPISIPSRNWAAFRGWSFTRLKTKETPSLGSGFDPYFVYSGSIPYLDGTFYLNHTFKKVSITFDSSVSWPGNDRLLTPNEFEIKRTVDGEGYNVAQCNMTKDWFLVQMLAHYNIGYQGFYVPEGYKDRMYSFFRNFQPMSRQVVDEVNYKDYQAVTLAYQHNNSGFVGYLAPTMRQGQPYPANYPYPLIGKSAVTSVTQKKFLCDRVMWRIPFSSNFMSMGALTDLGQNMLYANSAHALDMNFEVDPMDESTLLYVVFEVFDVVRVHQPHRGVIEAVYLRTPFSAGNATT

SEQ ID NO: 39 - protein, 942 aa, synthetic construct
MATPSMLPQWAYMHIAGQDASEYLSPGLVQFARATDTYFSLGNKFRNPTVAPTHDVTTDRSQRLTLRFVPVDREDNTYSYKVRYTLAVGDNRVLDMASTYFDIRGVLDRGPSFKPYSGTAYNSLAPKGAPNSSQWEQKKAGNGVTMETHTFGVAPMGGLNITIDGLQIGTNATANQNKPIYADKTFQPEPQVGEENWQETESFYGGRALKKDTSMKPCYGSYARPTNVKGGQAKLKVGADGVPTKEFDIDLAFFDTPGGTVNGQDEYKADIVMYTENTYLETPDTHVVYKPGKDDASSEINLVQQSMPNRPNYIGFRDNFIGLMYYNSTGNMGVLAGQASQLNAVVDLQDRNTELSYQLLLDSLGDRTRYFSMWNQAVDSYDPDVRIIENHGVEDELPNYCFPLDGSGTNAAYQGVKVKNGNNGNVQSQWENDDTVAARNQLCKGNIFAMEINLQANLWRSFLYSNVALYLPDSYKYTPANITLPTNTNTYDYMNGRVVPPSLVDAYINIGARWSLDPMDNVNPFNHHRNAGLRYRSMLLGNGRYVPFHIQVPQKFFAIKSLLLLPGSYTYEWNFRKDVNMILQSSLGNDLRTDGASISFTSINLYATFFPMAHNTASTLEAMLRNDTNDQSFNDYLSAANMLYPIPANATNVPISIPSRNWAAFRGWSFTRLKTKETPSLGSGFDPYFVYSGSIPYLDGTFYLNHTFKKVSITFDSSVSWPGNDRLLTPNEFEIKRTVDGEGYNVAQCNMTKDWFLVQMLAHYNIGYQGFYVPEGYKDRMYSFFRNFQPMSRQVVDEVNYKDYQAVTLAYQHNNSGFVGYLAPTMRQGQPYPANYPYPLIGKSAVTSVTQKKFLCDRVMWRIPFSSNFMSMGALTDLGQNMLYANSAHALDMNFEVDPMDESTLLYVVFEVFDVVRVHQPHRGVIEAVYLRTPFSAGNATT

SEQ ID NO: 40 - protein, 942 aa, synthetic construct
MATPSMLPQWAYMHIAGQDASEYLSPGLVQFARATDTYFSLGNKFRNPTVAPTHDVTTDRSQRLTLRFVPVDREDNTYSYKVRYTLAVGDNRVLDMASTYFDIRGVLDRGPSFKPYSGTAYNSLAPKGAPNSSQWEQKKAGNGDTMETHTFGVAPMGGENITIDGLQIGTNATANQNKPIYADKTFQPEPQVGEENWQETESFYGGRALKKDTSMKPCYGSYARPTNVKGGQAKLKVGADGVPTKEFDIDLAFFDTPGGTVNGQNEYKADIVMYTENTYLETPDTHVVYKPGKDDASSEINLVQQSMPNRPNYIGFRDNFIGLMYYNSTGNMGVLAGQASQLNAVVDLQDRNTELSYQLLLDSLGDRTRYFSMWNQAVDSYDPDVRIIENHGVEDELPNYCFPLDGSGTNAAYQGVKVKNGNNGNVQSQWENDDTVAARNQLCKGNIFAMEINLQANLWRSFLYSNVALYLPDSYKYTPANITLPTNTNTYDYMNGRVVPPSLVDAYINIGARWSLDPMDNVNPFNHHRNAGLRYRSMLLGNGRYVPFHIQVPQKFFAIKSLLLLPGSYTYEWNFRKDVNMILQSSLGNDLRTDGASISFTSINLYATFFPMAHNTASTLEAMLRNDTNDQSFNDYLSAANMLYPIPANATNVPISIPSRNWAAFRGWSFTRLKTKETPSLGSGFDPYFVYSGSIPYLDGTFYLNHTFKKVSITFDSSVSWPGNDRLLTPNEFEIKRTVDGEGYNVAQCNMTKDWFLVQMLAHYNIGYQGFYVPEGYKDRMYSFFRNFQPMSRQVVDEVNYKDYQAVTLAYQHNNSGFVGYLAPTMRQGQPYPANYPYPLIGKSAVTSVTQKKFLCDRVMWRIPFSSNFMSMGALTDLGQNMLYANSAHALDMNFEVDPMDESTLLYVVFEVFDVVRVHQPHRGVIEAVYLRTPFSAGNATT

SEQ ID NO: 41 - protein, 942 aa, synthetic construct
MATPSMLPQWAYMHIAGQDASEYLSPGLVQFARATDTYFSLGNKFRNPTVAPTHDVTTDRSQRLTLRFVPVDREDNTYSYKVRYTLAVGDNRVLDMASTYFDIRGVLDRGPSFKPYSGTAYNSLAPKGAPNSSQWEQKKAGNGVTMETHTFGVAPMGGLNITIDGLQIGTNATANQNKPIYADKTFQPEPQVGEENWQETESFYGGRALKKDTSMKPCYGSYARPTNVKGGQAKLKVGADGVPTKEFDIDLAFFDTPGGTVNGQNEYKADIVMYTENTYLETPDTHVVYKPGKDDASSEINLVQQSMPNRPNYIGFRDNFIGLMYYNSTGNMGVLAGQASQLNAVVDLQDRNTELSYQLLLDSLGDRTRYFSMWNQAVDSYDPDVRIIENHGVEDELPNYCFPLDGSGTNAAYQGVKVKNGNNGNVQSQWENDDTVAARNQLCKGNIFAMEINLQANLWRSFLYSNVALYLPDSYKYTPANITLPTNTNTYDYMNGRVVPPSLVDAYINIGARWSLDPMDNVNPFNHHRNAGLRYRSMLLGNGRYVPFHIQVPQKFFAIKSLLLLPGSYTYEWNFRKDVNMILQSSLGNDLRTDGASISFTSINLYATFFPMAHNTASTLEAMLRNDTNDQSFNDYLSAANMLYPIPANATNVPISIPSRNWAAFRGWSFTRLKTKETPSLGSGFDPYFVYSGSIPYLDGTFYLNHTFKKVSITFDSSVSWPGNDRLLTPNEFEIKRTVDGEGYNVAQCNMTKDWFLVQMLAHYNIGYQGFYVPEGYKDRMYSFFRNFQPMSRQVVDEVNYKDYQAVTLAYQHNNSGFVGYLAPTMRQGQPYPANYPYPLIGKSAVTSVTQKKFLCDRVMWRIPFSSNFMSMGALTDLGQNMLYANSAHALDMNFEVDPMDESTLLYVVFEVFDVVRVHQPHRGVIEAVYLRTPFSAGNATT

SEQ ID NO: 42 - protein, 942 aa, synthetic construct
MATPSMLPQWAYMHIAGQDASEYLSPGLVQFARATDTYFSLGNKFRNPTVAPTHDVTTDRSQRLTLRFVPVDREDNTYSYKVRYTLAVGDNRVLDMASTYFDIRGVLDRGPSFKPYSGTAYNSLAPKGAPNSSQWEQKKAGNGVTMETHTFGVAPMGGLNITIDGLQIGTNATANQNKPIYADKTFQPEPQVGEENWQETESFYGGRALKKDTSMKPCYGSYARPTNVKGGQAKLKVGADGVPTKEFDIDLAFFDTPGGTVNGQNEYKADIVMYTENTYLETPDTHVVYKPGKDDASSEINLVQQSMPNRPNYIGFRDNFIGLMYYNSTGNMGVLAGQASQLNAVVDLQDRNTELSYQLLLDSLGDRTRYFSMWNQAVDSYDPDVRIIENHGVEDELPNYCFPLDGSGTNAAYQGVKVKNGNVGVVLSLWENDDTVAARNQLCKGNIFAMEINLQANLWRSFLYSNVALYLPDSYKYTPANITLPTNTNTYDYMNGRVVPPSLVDAYINIGARWSLDPMDNVNPFNHHRNAGLRYRSMLLGNGRYVPFHIQVPQKFFAIKSLLLLPGSYTYEWNFRKDVNMILQSSLGNDLRTDGASISFTSINLYATFFPMAHNTASTLEAMLRNDTNDQSFNDYLSAANMLYPIPANATNVPISIPSRNWAAFRGWSFTRLKTKETPSLGSGFDPYFVYSGSIPYLDGTFYLNHTFKKVSITFDSSVSWPGNDRLLTPNEFEIKRTVDGEGYNVAQCNMTKDWFLVQMLAHYNIGYQGFYVPEGYKDRMYSFFRNFQPMSRQVVDEVNYKDYQAVTLAYQHNNSGFVGYLAPTMRQGQPYPANYPYPLIGKSAVTSVTQKKFLCDRVMWRIPFSSNFMSMGALTDLGQNMLYANSAHALDMNFEVDPMDESTLLYVVFEVFDVVRVHQPHRGVIEAVYLRTPFSAGNATT

SEQ ID NO: 43 - protein, 942 aa, synthetic construct
MATPSMLPQWAYMHIAGQDASEYLSPGLVQFARATDTYFSLGNKFRNPTVAPTHDVTTDRSQRLTLRFVPVDREDNTYSYKVRYTLAVGDNRVLDMASTYFDIRGVLDRGPSFKPYSGTAYNSLAPKGAPNSSQWEQKKAGNGVTMETHTFGVAPMGGLNITIDGLQIGTVATAVQVKPIYADKTFQPEPQVGEENWQETESFYGGRALKKDTSMKPCYGSYARPTNVKGGQAKLKVGADGVPTKEFDIDLAFFDTPGGTVNGQNEYKADIVMYTENTYLETPDTHVVYKPGKDDASSEINLVQQSMPNRPNYIGFRDNFIGLMYYNSTGNMGVLAGQASQLNAVVDLQDRNTELSYQLLLDSLGDRTRYFSMWNQAVDSYDPDVRIIENHGVEDELPNYCFPLDGSGTNAAYQGVKVKNGNNGNVQSQWENDDTVAARNQLCKGNIFAMEINLQANLWRSFLYSNVALYLPDSYKYTPANITLPTNTNTYDYMNGRVVPPSLVDAYINIGARWSLDPMDNVNPFNHHRNAGLRYRSMLLGNGRYVPFHIQVPQKFFAIKSLLLLPGSYTYEWNFRKDVNMILQSSLGNDLRTDGASISFTSINLYATFFPMAHNTASTLEAMLRNDTNDQSFNDYLSAANMLYPIPANATNVPISIPSRNWAAFRGWSFTRLKTKETPSLGSGFDPYFVYSGSIPYLDGTFYLNHTFKKVSITFDSSVSWPGNDRLLTPNEFEIKRTVDGEGYNVAQCNMTKDWFLVQMLAHYNIGYQGFYVPEGYKDRMYSFFRNFQPMSRQVVDEVNYKDYQAVTLAYQHNNSGFVGYLAPTMRQGQPYPANYPYPLIGKSAVTSVTQKKFLCDRVMWRIPFSSNFMSMGALTDLGQNMLYANSAHALDMNFEVDPMDESTLLYVVFEVFDVVRVHQPHRGVIEAVYLRTPFSAGNATT

SEQ ID NO: 44 - protein, 942 aa, synthetic construct
MATPSMLPQWAYMHIAGQDASEYLSPGLVQFARATDTYFSLGNKFRNPTVAPTHDVTTDRSQRLTLRFVPVDREDNTYSYKVRYTLAVGDNRVLDMASTYFDIRGVLDRGPSFKPYSGTAYNSLAPKGAPNSSQWEQKKAGNGVTMETHTFGVAPMGGLNITIDGLQIGTVATAVQVKPIYADKTFQPEPQVGEENWQETESFYGGRALKKDTSMKPCYGSYARPTNVKGGQAKLKVGADGVPTKEFDIDLAFFDTPGGTVNGQNEYKADIVMYTENTYLETPDTHVVYKPGKDDASSEINLVQQSMPNRPNYIGFRDNFIGLMYYNSTGNMGVLAGQASQLNAVVDLQDRNTELSYQLLLDSLGDRTRYFSMWNQAVDSYDPDVRIIENHGVEDELPNYCFPLDGSGTNAAYQGVKVKNGNVGVVLSLWENDDTVAARNQLCKGNIFAMEINLQANLWRSFLYSNVALYLPDSYKYTPANITLPTNTNTYDYMNGRVVPPSLVDAYINIGARWSLDPMDNVNPFNHHRNAGLRYRSMLLGNGRYVPFHIQVPQKFFAIKSLLLLPGSYTYEWNFRKDVNMILQSSLGNDLRTDGASISFTSINLYATFFPMAHNTASTLEAMLRNDTNDQSFNDYLSAANMLYPIPANATNVPISIPSRNWAAFRGWSFTRLKTKETPSLGSGFDPYFVYSGSIPYLDGTFYLNHTFKKVSITFDSSVSWPGNDRLLTPNEFEIKRTVDGEGYNVAQCNMTKDWFLVQMLAHYNIGYQGFYVPEGYKDRMYSFFRNFQPMSRQVVDEVNYKDYQAVTLAYQHNNSGFVGYLAPTMRQGQPYPANYPYPLIGKSAVTSVTQKKFLCDRVMWRIPFSSNFMSMGALTDLGQNMLYANSAHALDMNFEVDPMDESTLLYVVFEVFDVVRVHQPHRGVIEAVYLRTPFSAGNATT

SEQ ID NO: 45 - protein, 942 aa, synthetic construct
MATPSMLPQWAYMHIAGQDASEYLSPGLVQFARATDTYFSLGNKFRNPTVAPTHDVTTDRSQRLTLRFVPVDREDNTYSYKVRYTLAVGDNRVLDMASTYFDIRGVLDRGPSFKPYSGTAYNSLAPKGAPNSSQWEQKKAGNGVTMETHTFGVAPMGGLNITIDGLQIGTTATATQTKPIYADKTFQPEPQVGEENWQETESFYGGRALKKDTSMKPCYGSYARPTNVKGGQAKLKVGADGVPTKEFDIDLAFFDTPGGTVNGQNEYKADIVMYTENTYLETPDTHVVYKPGKDDASSEINLVQQSMPNRPNYIGFRDNFIGLMYYNSTGNMGVLAGQASQLNAVVDLQDRNTELSYQLLLDSLGDRTRYFSMWNQAVDSYDPDVRIIENHGVEDELPNYCFPLDGSGTNAAYQGVKVKNGNNGNVISIWENDDTVAARNQLCKGNIFAMEINLQANLWRSFLYSNVALYLPDSYKYTPANITLPTNTNTYDYMNGRVVPPSLVDAYINIGARWSLDPMDNVNPFNHHRNAGLRYRSMLLGNGRYVPFHIQVPQKFFAIKSLLLLPGSYTYEWNFRKDVNMILQSSLGNDLRTDGASISFTSINLYATFFPMAHNTASTLEAMLRNDTNDQSFNDYLSAANMLYPIPANATNVPISIPSRNWAAFRGWSFTRLKTKETPSLGSGFDPYFVYSGSIPYLDGTFYLNHTFKKVSITFDSSVSWPGNDRLLTPNEFEIKRTVDGEGYNVAQCNMTKDWFLVQMLAHYNIGYQGFYVPEGYKDRMYSFFRNFQPMSRQVVDEVNYKDYQAVTLAYQHNNSGFVGYLAPTMRQGQPYPANYPYPLIGKSAVTSVTQKKFLCDRVMWRIPFSSNFMSMGALTDLGQNMLYANSAHALDMNFEVDPMDESTLLYVVFEVFDVVRVHQPHRGVIEAVYLRTPFSAGNATT

SEQ ID NO: 46 - protein, 942 aa, synthetic construct
MATPSMLPQWAYMHIAGQDASEYLSPGLVQFARATDTYFSLGNKFRNPTVAPTHDVTTDRSQRLTLRFVPVDREDNTYSYKVRYTLAVGDNRVLDMASTYFDIRGVLDRGPSFKPYSGTAYNSLAPKGAPNSSQWEQKKAGNGVTMETHTFGVAPMGGLNITIDGLQIGTTATATQTKPIYADKTFQPEPQVGEENWQETESFYGGRALKKDTSMKPCYGSYARPTNVKGGQAKLKVGADGVPTKEFDIDLAFFDTPGGTVNGQNEYKADIVMYTENTYLETPDTHVVYKPGKDDASSEINLVQQSMPNRPNYIGFRDNFIGLMYYNSTGNMGVLAGQASQLNAVVDLQDRNTELSYQLLLDSLGDRTRYFSMWNQAVDSYDPDVRIIENHGVEDELPNYCFPLDGSGTNAAYQGVKVKNGNVGVVISIWENDDTVAARNQLCKGNIFAMEINLQANLWRSFLYSNVALYLPDSYKYTPANITLPTNTNTYDYMNGRVVPPSLVDAYINIGARWSLDPMDNVNPFNHHRNAGLRYRSMLLGNGRYVPFHIQVPQKFFAIKSLLLLPGSYTYEWNFRKDVNMILQSSLGNDLRTDGASISFTSINLYATFFPMAHNTASTLEAMLRNDTNDQSFNDYLSAANMLYPIPANATNVPISIPSRNWAAFRGWSFTRLKTKETPSLGSGFDPYFVYSGSIPYLDGTFYLNHTFKKVSITFDSSVSWPGNDRLLTPNEFEIKRTVDGEGYNVAQCNMTKDWFLVQMLAHYNIGYQGFYVPEGYKDRMYSFFRNFQPMSRQVVDEVNYKDYQAVTLAYQHNNSGFVGYLAPTMRQGQPYPANYPYPLIGKSAVTSVTQKKFLCDRVMWRIPFSSNFMSMGALTDLGQNMLYANSAHALDMNFEVDPMDESTLLYVVFEVFDVVRVHQPHRGVIEAVYLRTPFSAGNATT

SEQ ID NO: 47 - protein, 942 aa, synthetic construct
MATPSMLPQWAYMHIAGQDASEYLSPGLVQFARATDTYFSLGNKFRNPTVAPTHDVTTDRSQRLTLRFVPVDREDNTYSYKVRYTLAVGDNRVLDMASTYFDIRGVLDRGPSFKPYSGTAYNSLAPKGAPNSSQWEQKKAGNGVTMETHTFGVAPMGGLNITIDGLQIGTVATAVQVKPIYADKTFQPEPQVGEENWQETESFYGGRALKKDTSMKPCYGSYARPTNVKGGQAKLKVGADGVPTKEFDIDLAFFDTPGGTVNGQNEYKADIVMYTENTYLETPDTHVVYKPGKDDASSEINLVQQSMPNRPNYIGFRDNFIGLMYYNSTGNMGVLAGQASQLNAVVDLQDRNTELSYQLLLDSLGDRTRYFSMWNQAVDSYDPDVRIIENHGVEDELPNYCFPLDGSGTNAAYQGVKVKNGNNGNVISIWENDDTVAARNQLCKGNIFAMEINLQANLWRSFLYSNVALYLPDSYKYTPANITLPTNTNTYDYMNGRVVPPSLVDAYINIGARWSLDPMDNVNPFNHHRNAGLRYRSMLLGNGRYVPFHIQVPQKFFAIKSLLLLPGSYTYEWNFRKDVNMILQSSLGNDLRTDGASISFTSINLYATFFPMAHNTASTLEAMLRNDTNDQSFNDYLSAANMLYPIPANATNVPISIPSRNWAAFRGWSFTRLKTKETPSLGSGFDPYFVYSGSIPYLDGTFYLNHTFKKVSITFDSSVSWPGNDRLLTPNEFEIKRTVDGEGYNVAQCNMTKDWFLVQMLAHYNIGYQGFYVPEGYKDRMYSFFRNFQPMSRQVVDEVNYKDYQAVTLAYQHNNSGFVGYLAPTMRQGQPYPANYPYPLIGKSAVTSVTQKKFLCDRVMWRIPFSSNFMSMGALTDLGQNMLYANSAHALDMNFEVDPMDESTLLYVVFEVFDVVRVHQPHRGVIEAVYLRTPFSAGNATT

SEQ ID NO: 48 - protein, 942 aa, synthetic construct
MATPSMLPQWAYMHIAGQDASEYLSPGLVQFARATDTYFSLGNKFRNPTVAPTHDVTTDRSQRLTLRFVPVDREDNTYSYKVRYTLAVGDNRVLDMASTYFDIRGVLDRGPSFKPYSGTAYNSLAPKGAPNSSQWEQKKAGNGVTMETHTFGVAPMGGLNITIDGLQIGTVATAVQVKPIYADKTFQPEPQVGEENWQETESFYGGRALKKDTSMKPCYGSYARPTNVKGGQAKLKVGADGVPTKEFDIDLAFFDTPGGTVNGQNEYKADIVMYTENTYLETPDTHVVYKPGKDDASSEINLVQQSMPNRPNYIGFRDNFIGLMYYNSTGNMGVLAGQASQLNAVVDLQDRNTELSYQLLLDSLGDRTRYFSMWNQAVDSYDPDVRIIENHGVEDELPNYCFPLDGSGTNAAYQGVKVKNGNVGVVISIWENDDTVAARNQLCKGNIFAMEINLQANLWRSFLYSNVALYLPDSYKYTPANITLPTNTNTYDYMNGRVVPPSLVDAYINIGARWSLDPMDNVNPFNHHRNAGLRYRSMLLGNGRYVPFHIQVPQKFFAIKSLLLLPGSYTYEWNFRKDVNMILQSSLGNDLRTDGASISFTSINLYATFFPMAHNTASTLEAMLRNDTNDQSFNDYLSAANMLYPIPANATNVPISIPSRNWAAFRGWSFTRLKTKETPSLGSGFDPYFVYSGSIPYLDGTFYLNHTFKKVSITFDSSVSWPGNDRLLTPNEFEIKRTVDGEGYNVAQCNMTKDWFLVQMLAHYNIGYQGFYVPEGYKDRMYSFFRNFQPMSRQVVDEVNYKDYQAVTLAYQHNNSGFVGYLAPTMRQGQPYPANYPYPLIGKSAVTSVTQKKFLCDRVMWRIPFSSNFMSMGALTDLGQNMLYANSAHALDMNFEVDPMDESTLLYVVFEVFDVVRVHQPHRGVIEAVYLRTPFSAGNATT

SEQ ID NO: 49 - protein, 942 aa, synthetic construct
MATPSMLPQWAYMHIAGQDASEYLSPGLVQFARATDTYFSLGNKFRNPTVAPTHDVTTDRSQRLTLRFVPVDREDNTYSYKVRYTLAVGDNRVLDMASTYFDIRGVLDRGPSFKPYSGTAYNSLAPKGAPNSSQWEQKKAGNGVTMETHTFGVAPMGGLNITIDGLQIGTNATANQNKPIYADKTFQPEPQVGEENWQETESFYGGRALKKDTSMKPCYGSYARPTNVKGGQAKLKVGADGVPTKEFDIDLAFFDTPGGTVNGQNEYKADIVMYTENTYLETPDTHVVYKPGKDDASSEINLVQQSMPNRPNYIGFRDNFIGLMYYNSTGNMGVLAGQASQLNAVVDLQDRNTELSYQLLLDSLGDRTRYFSMWNQAVDSYDPDVRIIENHGVEDELPNYCFPLDGSGTNAAYQGVKVKNGNNGNVISIWENDDTVAARNQLCKGNIFAMEINLQANLWRSFLYSNVALYLPDSYKYTPANITLPTNTNTYDYMNGRVVPPSLVDAYINIGARWSLDPMDNVNPFNHHRNAGLRYRSMLLGNGRYVPFHIQVPQKFFAIKSLLLLPGSYTYEWNFRKDVNMILQSSLGNDLRTDGASISFTSINLYATFFPMAHNTASTLEAMLRNDTNDQSFNDYLSAANMLYPIPANATNVPISIPSRNWAAFRGWSFTRLKTKETPSLGSGFDPYFVYSGSIPYLDGTFYLNHTFKKVSITFDSSVSWPGNDRLLTPNEFEIKRTVDGEGYNVAQCNMTKDWFLVQMLAHYNIGYQGFYVPEGYKDRMYSFFRNFQPMSRQVVDEVNYKDYQAVTLAYQHNNSGFVGYLAPTMRQGQPYPANYPYPLIGKSAVTSVTQKKFLCDRVMWRIPFSSNFMSMGALTDLGQNMLYANSAHALDMNFEVDPMDESTLLYVVFEVFDVVRVHQPHRGVIEAVYLRTPFSAGNATT

SEQ ID NO: 50 - protein, 942 aa, synthetic construct
MATPSMLPQWAYMHIAGQDASEYLSPGLVQFARATDTYFSLGNKFRNPTVAPTHDVTTDRSQRLTLRFVPVDREDNTYSYKVRYTLAVGDNRVLDMASTYFDIRGVLDRGPSFKPYSGTAYNSLAPKGAPNSSQWEQKKAGNGVTMETHTFGVAPMGGLNITIDGLQIGTNATANQNKPIYADKTFQPEPQVGEENWQETESFYGGRALKKDTSMKPCYGSYARPTNVKGGQAKLKVGADGVPTKEFDIDLAFFDTPGGTVNGQNEYKADIVMYTENTYLETPDTHVVYKPGKDDASSEINLVQQSMPNRPNYIGFRDNFIGLMYYNSTGNMGVLAGQASQLNAVVDLQDRNTELSYQLLLDSLGDRTRYFSMWNQAVDSYDPDVRIIENHGVEDELPNYCFPLDGSGTNAAYQGVKVKNGNVGVVISIWENDDTVAARNQLCKGNIFAMEINLQANLWRSFLYSNVALYLPDSYKYTPANITLPTNTNTYDYMNGRVVPPSLVDAYINIGARWSLDPMDNVNPFNHHRNAGLRYRSMLLGNGRYVPFHIQVPQKFFAIKSLLLLPGSYTYEWNFRKDVNMILQSSLGNDLRTDGASISFTSINLYATFFPMAHNTASTLEAMLRNDTNDQSFNDYLSAANMLYPIPANATNVPISIPSRNWAAFRGWSFTRLKTKETPSLGSGFDPYFVYSGSIPYLDGTFYLNHTFKKVSITFDSSVSWPGNDRLLTPNEFEIKRTVDGEGYNVAQCNMTKDWFLVQMLAHYNIGYQGFYVPEGYKDRMYSFFRNFQPMSRQVVDEVNYKDYQAVTLAYQHNNSGFVGYLAPTMRQGQPYPANYPYPLIGKSAVTSVTQKKFLCDRVMWRIPFSSNFMSMGALTDLGQNMLYANSAHALDMNFEVDPMDESTLLYVVFEVFDVVRVHQPHRGVIEAVYLRTPFSAGNATT